European Patent Application EP 4 202 058 A1, published June 28, 2023. Title: Element, Kit and Library Construction Method Compatible With Double Sequencing Platforms. Applicant: NANODIGMBIO(NANJING) BIOTECHNOLOGY CO., LTD. The sequence listing filed with the application follows.

SEQUENCE LISTING (852 sequences)

SEQ ID NO: 1 - DNA, 59 bp, Artificial Sequence
  Synthesied
  misc_feature (1)..(1): 5'phosphorlation
  misc_feature (30)..(39): P5-index(selected from one of Table 1-1)
aatgatacggcgaccaccgagatctacacnnnnnnnnnnacactctttccctacacgac

SEQ ID NO: 2 - DNA, 55 bp, Artificial Sequence
  Synthesied
  misc_feature (25)..(34): p7-index(selected from one of Table 1-2)
caagcagaagacggcatacgagatnnnnnnnnnngtgactggagttcagacgtgt

SEQ ID NO: 3 - DNA, 72 bp, Artificial Sequence
  Synthesied
  misc_feature (1)..(1): 5'phosphorlation
  misc_feature (30)..(39): P5-index
  misc_feature (72)..(72): phosphorothioate
aatgatacggcgaccaccgagatctacacnnnnnnnnnnacactctttccctacacgacgctcttccgatct

SEQ ID NO: 4 - DNA, 67 bp, Artificial Sequence
  Synthesied
  misc_feature (1)..(1): 5'phosphorlation
  misc_feature (34)..(43): P7-index
gatcggaagagcacacgtctgaactccagtcacnnnnnnnnnnatctcgtatgccgtcttctgcttg

SEQ ID NO: 5 - DNA, 23 bp, Artificial Sequence
  Synthesied
  misc_feature (1)..(1): 5'phosphorlation
aatgatacggcgaccaccgagat

SEQ ID NO: 6 - DNA, 21 bp, Artificial Sequence
  Synthesied
  misc_feature (1)..(21): same with Illumina P7 primer
caagcagaagacggcatacga

SEQ ID NO: 7 - DNA, 33 bp, Artificial Sequence
  Synthesied
  misc_feature (33)..(33): phosphorothioate
acactctttccctacacgacgctcttccgatct

SEQ ID NO: 8 - DNA, 33 bp, Artificial Sequence
  Synthesied
  misc_feature (1)..(1): 5'phosphorlation
gatcggaagagcacacgtctgaactccagtcac

SEQ ID NO: 9 - DNA, 10 bp, Artificial Sequence
  Synthesied
  misc_feature (1)..(10): P5-index
gtgataagca

SEQ ID NO: 10 - DNA, 10 bp, Artificial Sequence
  Synthesied
  misc_feature (1)..(10): P5-index
tcctattagg

SEQ ID NO: 11 - DNA, 10 bp, Artificial Sequence
  Synthesied
  misc_feature (1)..(10): P5-index
catggcgtac

SEQ ID NO: 12 - DNA, 10 bp, Artificial Sequence
  Synthesied
  misc_feature (1)..(10): P5-index
agaccgcctt

SEQ ID NO: 13 - DNA, 10 bp, Artificial Sequence
  Synthesied
  misc_feature (1)..(10): P5-index
cgtgccgatt

SEQ ID NO: 14 - DNA, 10 bp, Artificial Sequence
  Synthesied
  misc_feature (1)..(10): P5-index
ttcaggtggc

SEQ ID NO: 15 - DNA, 10 bp, Artificial Sequence
  Synthesied
  misc_feature (1)..(10): P5-index
aagttactcg

SEQ ID NO: 16 - DNA, 10 bp, Artificial Sequence
  Synthesied
  misc_feature (1)..(10): P5-index
gcacatacaa

SEQ ID NO: 17 - DNA, 10 bp, Artificial Sequence
  Synthesied
  misc_feature (1)..(10): P5-index
ggactgtgga

SEQ ID NO: 18 - DNA, 10 bp, Artificial Sequence
  Synthesied
  misc_feature (1)..(10): P5-index
cctaataacg

SEQ ID NO: 19 - DNA, 10 bp, Artificial Sequence
  Synthesied
  misc_feature (1)..(10): P5-index
aaggcactat

SEQ ID NO: 20 - DNA, 10 bp, Artificial Sequence
  Synthesied
  misc_feature (1)..(10): P5-index
ttctgcgctc

SEQ ID NO: 21 - DNA, 10 bp, Artificial Sequence
  Synthesied
  misc_feature (1)..(10): P5-index
gctctgcttc

SEQ ID NO: 22 - DNA, 10 bp, Artificial Sequence
  Synthesied
  misc_feature (1)..(10): P5-index
tagtcatacg

SEQ ID NO: 23 - DNA, 10 bp, Artificial Sequence
  Synthesied
  misc_feature (1)..(10): P5-index
ctaagtacga

SEQ ID NO: 24 - DNA, 10 bp, Artificial Sequence
  Synthesied
  misc_feature (1)..(10): P5-index
agcgacggat

SEQ ID NO: 25 - DNA, 10 bp, Artificial Sequence
  Synthesied
  misc_feature (1)..(10): P5-index
cgaggcgaat

SEQ ID NO: 26 - DNA, 10 bp, Artificial Sequence
  Synthesied
  misc_feature (1)..(10): P5-index
tagccgcttg

SEQ ID NO: 27 - DNA, 10 bp, Artificial Sequence
  Synthesied
  misc_feature (1)..(10): P5-index
gttaatagcc

SEQ ID NO: 28 - DNA, 10 bp, Artificial Sequence
  Synthesied
  misc_feature (1)..(10): P5-index
accttatcga

SEQ ID NO: 29 - DNA, 10 bp, Artificial Sequence
  Synthesied
  misc_feature (1)..(10): P5-index
ccagattcgt

SEQ ID NO: 30 - DNA, 10 bp, Artificial Sequence
  Synthesied
  misc_feature (1)..(10): P5-index
ttgatccgca

SEQ ID NO: 31 - DNA, 10 bp, Artificial Sequence
  Synthesied
  misc_feature (1)..(10): P5-index
gactgaatag

SEQ ID NO: 32 - DNA, 10 bp, Artificial Sequence
  Synthesied
  misc_feature (1)..(10): P5-index
agtccggatc

SEQ ID NO: 33 - DNA, 10 bp, Artificial Sequence
  Synthesied
  misc_feature (1)..(10): P5-index
gtcggctgta

SEQ ID NO: 34 - DNA, 10 bp, Artificial Sequence
  Synthesied
  misc_feature (1)..(10): P5-index
tgatcaatgc

SEQ ID NO: 35 - DNA, 10 bp, Artificial Sequence
  Synthesied
  misc_feature (1)..(10): P5-index
actaatgccg

SEQ ID NO: 36 - DNA, 10 bp, Artificial Sequence
  Synthesied
  misc_feature (1)..(10): P5-index
cagctgcaat

SEQ ID NO: 37 - DNA, 10 bp, Artificial Sequence
  Synthesied
  misc_feature (1)..(10): P5-index
cggcaaggat

SEQ ID NO: 38 - DNA, 10 bp, Artificial Sequence
  Synthesied
  misc_feature (1)..(10): P5-index
aatatgtcgc

SEQ ID NO: 39 - DNA, 10 bp, Artificial Sequence
  Synthesied
  misc_feature (1)..(10): P5-index
ttatgccaca

SEQ ID NO: 40 - DNA, 10 bp, Artificial Sequence
  Synthesied
  misc_feature (1)..(10): P5-index
gccgctattg

SEQ ID NO: 41 - DNA, 10 bp, Artificial Sequence
  Synthesied
  misc_feature (1)..(10): P5-index
cgtacctgtg

SEQ ID NO: 42 - DNA, 10 bp, Artificial Sequence
  Synthesied
  misc_feature (1)..(10): P5-index
gcatataagc

SEQ ID NO: 43 - DNA, 10 bp, Artificial Sequence
  Synthesied
  misc_feature (1)..(10): P5-index
aaggtagtct

SEQ ID NO: 44 - DNA, 10 bp, Artificial Sequence
  Synthesied
  misc_feature (1)..(10): P5-index
ttccggccaa

SEQ ID NO: 45 - DNA, 10 bp, Artificial Sequence
  Synthesied
  misc_feature (1)..(10): P5-index
ggcatagcga

SEQ ID NO: 46 - DNA, 10 bp, Artificial Sequence
  Synthesied
  misc_feature (1)..(10): P5-index
taggctaact

SEQ ID NO: 47 - DNA, 10 bp, Artificial Sequence
  Synthesied
  misc_feature (1)..(10): P5-index
acatagtgac

SEQ ID NO: 48 - DNA, 10 bp, Artificial Sequence
  Synthesied
  misc_feature (1)..(10): P5-index
cttcgccttg

SEQ ID NO: 49 - DNA, 10 bp, Artificial Sequence
  Synthesied
  misc_feature (1)..(10): P5-index
gagtgcacga

SEQ ID NO: 50 - DNA, 10 bp, Artificial Sequence
  Synthesied
  misc_feature (1)..(10): P5-index
tgcgaattct

SEQ ID NO: 51 - DNA, 10 bp, Artificial Sequence
  Synthesied
  misc_feature (1)..(10): P5-index
ccaatggaag

SEQ ID NO: 52 - DNA, 10 bp, Artificial Sequence
  Synthesied
  misc_feature (1)..(10): P5-index
attcctcgtc

SEQ ID NO: 53 - DNA, 10 bp, Artificial Sequence
  Synthesied
  misc_feature (1)..(10): P5-index
gatgtgtgaa

SEQ ID NO: 54 - DNA, 10 bp, Artificial Sequence
  Synthesied
  misc_feature (1)..(10): P5-index
atgcacaatg

SEQ ID NO: 55 - DNA, 10 bp, Artificial Sequence
  Synthesied
  misc_feature (1)..(10): P5-index
tcaagagcgc

SEQ ID NO: 56 - DNA, 10 bp, Artificial Sequence
  Synthesied
  misc_feature (1)..(10): P5-index
cgctctctct

SEQ ID NO: 57 - DNA, 10 bp, Artificial Sequence
  Synthesied
  misc_feature (1)..(10): P5-index
cgaatatacc

SEQ ID NO: 58 - DNA, 10 bp, Artificial Sequence
  Synthesied
  misc_feature (1)..(10): P5-index
tacgccggaa

SEQ ID NO: 59 - DNA, 10 bp, Artificial Sequence
  Synthesied
  misc_feature (1)..(10): P5-index
gcttatatgg

SEQ ID NO: 60 - DNA, 10 bp, Artificial Sequence
  Synthesied
  misc_feature (1)..(10): P5-index
atgcggcctt

SEQ ID NO: 61 - DNA, 10 bp, Artificial Sequence
  Synthesied
  misc_feature (1)..(10): P5-index
ggttcgtcac

SEQ ID NO: 62 - DNA, 10 bp, Artificial Sequence
  Synthesied
  misc_feature (1)..(10): P5-index
tagaatgtgg

SEQ ID NO: 63 - DNA, 10 bp, Artificial Sequence
  Synthesied
  misc_feature (1)..(10): P5-index
ccagtaagta

SEQ ID NO: 64 - DNA, 10 bp, Artificial Sequence
  Synthesied
  misc_feature (1)..(10): P5-index
atccgccact

SEQ ID NO: 65 - DNA, 10 bp, Artificial Sequence
  Synthesied
  misc_feature (1)..(10): P5-index
agatcacacc

SEQ ID NO: 66 - DNA, 10 bp, Artificial Sequence
  Synthesied
  misc_feature (1)..(10): P5-index
gccgtgataa

SEQ ID NO: 67 - DNA, 10 bp, Artificial Sequence
  Synthesied
  misc_feature (1)..(10): P5-index
cataatgcgt

SEQ ID NO: 68 - DNA, 10 bp, Artificial Sequence
  Synthesied
  misc_feature (1)..(10): P5-index
ttgcgctgtg

SEQ ID NO: 69 - DNA, 10 bp, Artificial Sequence
  Synthesied
  misc_feature (1)..(10): P5-index
gtatagttgc

SEQ ID NO: 70 - DNA, 10 bp, Artificial Sequence
  Synthesied
  misc_feature (1)..(10): P5-index
tccactagat

SEQ ID NO: 71 - DNA, 10 bp, Artificial Sequence
  Synthesied
  misc_feature (1)..(10): P5-index
cgtgtagctg

SEQ ID NO: 72 - DNA, 10 bp, Artificial Sequence
  Synthesied
  misc_feature (1)..(10): P5-index
aagcgccaca

SEQ ID NO: 73 - DNA, 10 bp, Artificial Sequence
  Synthesied
  misc_feature (1)..(10): P5-index
agaggtgcgt

SEQ ID NO: 74 - DNA, 10 bp, Artificial Sequence
  Synthesied
  misc_feature (1)..(10): P5-index
ttgtcaagac

SEQ ID NO: 75 - DNA, 10 bp, Artificial Sequence
  Synthesied
  misc_feature (1)..(10): P5-index
cctaaccata

SEQ ID NO: 76 - DNA, 10 bp, Artificial Sequence
  Synthesied
  misc_feature (1)..(10): P5-index
gacctgttcg

SEQ ID NO: 77 - DNA, 10 bp, Artificial Sequence
  Synthesied
  misc_feature (1)..(10): P5-index
cctctagcac

SEQ ID NO: 78 - DNA, 10 bp, Artificial Sequence
  Synthesied
  misc_feature (1)..(10): P5-index
gaatatctgg

SEQ ID NO: 79 - DNA, 10 bp, Artificial Sequence
  Synthesied
  misc_feature (1)..(10): P5-index
tgcaggaata

SEQ ID NO: 80 - DNA, 10 bp, Artificial Sequence
  Synthesied
  misc_feature (1)..(10): P5-index
atggcctgct

SEQ ID NO: 81 - DNA, 10 bp, Artificial Sequence
  Synthesied
  misc_feature (1)..(10): P5-index
atgcagcgga

SEQ ID NO: 82 - DNA, 10 bp, Artificial Sequence
  Synthesied
  misc_feature (1)..(10): P5-index
tatagatccg

SEQ ID NO: 83 - DNA, 10 bp, Artificial Sequence
  Synthesied
  misc_feature (1)..(10): P5-index
ggcttcaatt

SEQ ID NO: 84 - DNA, 10 bp, Artificial Sequence
  Synthesied
  misc_feature (1)..(10): P5-index
ccagctgtac

SEQ ID NO: 85 - DNA, 10 bp, Artificial Sequence
  Synthesied
  misc_feature (1)..(10): P5-index
ccacggtgtt

SEQ ID NO: 86 - DNA, 10 bp, Artificial Sequence
  Synthesied
  misc_feature (1)..(10): P5-index
gagaataagg

SEQ ID NO: 87 - DNA, 10 bp, Artificial Sequence
  Synthesied
  misc_feature (1)..(10): P5-index
tgtgccgcaa

SEQ ID NO: 88 - DNA, 10 bp, Artificial Sequence
  Synthesied
  misc_feature (1)..(10): P5-index
atcttactcc

SEQ ID NO: 89 - DNA, 10 bp, Artificial Sequence
  Synthesied
  misc_feature (1)..(10): P5-index
gctgcagcat

SEQ ID NO: 90 - DNA, 10 bp, Artificial Sequence
  Synthesied
  misc_feature (1)..(10): P5-index
caatattgcc

SEQ ID NO: 91 - DNA, 10 bp, Artificial Sequence
  Synthesied
  misc_feature (1)..(10): P5-index
atgatgatgg

SEQ ID NO: 92 - DNA, 10 bp, Artificial Sequence
  Synthesied
  misc_feature (1)..(10): P5-index
tgccgccata

SEQ ID NO: 93 - DNA, 10 bp, Artificial Sequence
  Synthesied
  misc_feature (1)..(10): P5-index
tctctgtgtg

SEQ ID NO: 94 - DNA, 10 bp, Artificial Sequence
  Synthesied
  misc_feature (1)..(10): P5-index
cggtgaacaa

SEQ ID NO: 95 - DNA, 10 bp, Artificial Sequence
  Synthesied
  misc_feature (1)..(10): P5-index
gaagatcagt

SEQ ID NO: 96 - DNA, 10 bp, Artificial Sequence
  Synthesied
  misc_feature (1)..(10): P5-index
atcaccgtcc

SEQ ID NO: 97 - DNA, 10 bp, Artificial Sequence
  Synthesied
  misc_feature (1)..(10): P5-index
tgctagaggc

SEQ ID NO: 98 - DNA, 10 bp, Artificial Sequence
  Synthesied
  misc_feature (1)..(10): P5-index
catgttgtca

SEQ ID NO: 99 - DNA, 10 bp, Artificial Sequence
  Synthesied
  misc_feature (1)..(10): P5-index
ataagccaag

SEQ ID NO: 100 - DNA, 10 bp, Artificial Sequence
  Synthesied
  misc_feature (1)..(10): P5-index
gcgccatctt

SEQ ID NO: 101 - DNA, 10 bp, Artificial Sequence
  Synthesied
  misc_feature (1)..(10): P5-index
ttccgaacgc

SEQ ID NO: 102 - DNA, 10 bp, Artificial Sequence
  Synthesied
  misc_feature (1)..(10): P5-index
ggaacttaag

SEQ ID NO: 103 - DNA, 10 bp, Artificial Sequence
  Synthesied
  misc_feature (1)..(10): P5-index
cattagctct

SEQ ID NO: 104 - DNA, 10 bp, Artificial Sequence
  Synthesied
  misc_feature (1)..(10): P5-index
acggtcggta

SEQ ID NO: 105 - DNA, 10 bp, Artificial Sequence
  Synthesied
  misc_feature (1)..(10): P5-index
cttgtggcca

SEQ ID NO: 106 - DNA, 10 bp, Artificial Sequence
  Synthesied
  misc_feature (1)..(10): P5-index
aagaacatgc

SEQ ID NO: 107 - DNA, 10 bp, Artificial Sequence
  Synthesied
  misc_feature (1)..(10): P5-index
ggctgatatt

SEQ ID NO: 108 - DNA, 10 bp, Artificial Sequence
  Synthesied
  misc_feature (1)..(10): P5-index
tcacctcgag

SEQ ID NO: 109 - DNA, 10 bp, Artificial Sequence
  Synthesied
  misc_feature (1)..(10): P5-index
ccattcatag

SEQ ID NO: 110 - DNA, 10 bp, Artificial Sequence
  Synthesied
  misc_feature (1)..(10): P5-index
aaggaggcga

SEQ ID NO: 111 - DNA, 10 bp, Artificial Sequence
  Synthesied
  misc_feature (1)..(10): P5-index
ttcacacatc

SEQ ID NO: 112 - DNA, 10 bp, Artificial Sequence
  Synthesied
  misc_feature (1)..(10): P5-index
ggtcgttgct

SEQ ID NO: 113 - DNA, 10 bp, Artificial Sequence
  Synthesied
  misc_feature (1)..(10): P5-index
ccacgcagaa

SEQ ID NO: 114 - DNA, 10 bp, Artificial Sequence
  Synthesied
  misc_feature (1)..(10): P5-index
aagtcatcct

SEQ ID NO: 115 - DNA, 10 bp, Artificial Sequence
  Synthesied
  misc_feature (1)..(10): P5-index
ttcatgcatg

SEQ ID NO: 116 - DNA, 10 bp, Artificial Sequence
  Synthesied
  misc_feature (1)..(10): P5-index
ggtgatgtgc

SEQ ID NO: 117 - DNA, 10 bp, Artificial Sequence
  Synthesied
  misc_feature (1)..(10): P5-index
cctatccgtg

SEQ ID NO: 118 - DNA, 10 bp, Artificial Sequence
  Synthesied
  misc_feature (1)..(10): P5-index
aagtgtgacc

SEQ ID NO: 119 - DNA, 10 bp, Artificial Sequence
  Synthesied
  misc_feature (1)..(10): P5-index
ttagcgatga

SEQ ID NO: 120 - DNA, 10 bp, Artificial Sequence
  Synthesied
  misc_feature (1)..(10): P5-index
ggccaatcat

SEQ ID NO: 121 - DNA, 10 bp, Artificial Sequence
  Synthesied
  misc_feature (1)..(10): P5-index
cgctaagacc

SEQ ID NO: 122 - DNA, 10 bp, Artificial Sequence
  Synthesied
  misc_feature (1)..(10): P5-index
aatccgtctt

SEQ ID NO: 123 - DNA, 10 bp, Artificial Sequence
  Synthesied
  misc_feature (1)..(10): P5-index
ttagtcctgg

SEQ ID NO: 124 - DNA, 10 bp, Artificial Sequence
  Synthesied
  misc_feature (1)..(10): P5-index
gcgagtagaa

SEQ ID NO: 125 - DNA, 10 bp, Artificial Sequence
  Synthesied
  misc_feature (1)..(10): P5-index
tgaggattcg

SEQ ID NO: 126 - DNA, 10 bp, Artificial Sequence
  Synthesied
  misc_feature (1)..(10): P5-index
aatcctggaa

SEQ ID NO: 127 - DNA, 10 bp, Artificial Sequence
  Synthesied
  misc_feature (1)..(10): P5-index
ccgaagcatt

SEQ ID NO: 128 - DNA, 10 bp, Artificial Sequence
  Synthesied
  misc_feature (1)..(10): P5-index
gtcttcacgc

SEQ ID NO: 129 - DNA, 10 bp, Artificial Sequence
  Synthesied
  misc_feature (1)..(10): P5-index
cagtcggcat

SEQ ID NO: 130 - DNA, 10 bp, Artificial Sequence
  Synthesied
  misc_feature (1)..(10): P5-index
accagacata

SEQ ID NO: 131 - DNA, 10 bp, Artificial Sequence
  Synthesied
  misc_feature (1)..(10): P5-index
ttagactgcc

SEQ ID NO: 132 - DNA, 10 bp, Artificial Sequence
  Synthesied
  misc_feature (1)..(10): P5-index
ggtcttatgg

SEQ ID NO: 133 - DNA, 10 bp, Artificial Sequence
  Synthesied
  misc_feature (1)..(10): P5-index
gacggtgatc

SEQ ID NO: 134 - DNA, 10 bp, Artificial Sequence
  Synthesied
  misc_feature (1)..(10): P5-index
acgttcctaa

SEQ ID NO: 135 - DNA, 10 bp, Artificial Sequence
  Synthesied
  misc_feature (1)..(10): P5-index
ctaacaagct

SEQ ID NO: 136 - DNA, 10 bp, Artificial Sequence
  Synthesied
  misc_feature (1)..(10): P5-index
tgtcagtcgg

SEQ ID NO: 137 - DNA, 10 bp, Artificial Sequence
  Synthesied
  misc_feature (1)..(10): P5-index
tagcgacctc

SEQ ID NO: 138 - DNA, 10 bp, Artificial Sequence
  Synthesied
  misc_feature (1)..(10): P5-index
actgagaaca

SEQ ID NO: 139 - DNA, 10 bp, Artificial Sequence
  Synthesied
  misc_feature (1)..(10): P5-index
gtatcttggt

SEQ ID NO: 140 - DNA, 10 bp, Artificial Sequence
  Synthesied
  misc_feature (1)..(10): P5-index
cgcatcgtag

SEQ ID NO: 141 - DNA, 10 bp, Artificial Sequence
  Synthesied
  misc_feature (1)..(10): P5-index
catccttacg

SEQ ID NO: 142 - DNA, 10 bp, Artificial Sequence
  Synthesied
  misc_feature (1)..(10): P5-index
aggtagagac

SEQ ID NO: 143 - DNA, 10 bp, Artificial Sequence
  Synthesied
  misc_feature (1)..(10): P5-index
ttcgtagcgt

SEQ ID NO: 144 - DNA, 10 bp, Artificial Sequence
  Synthesied
  misc_feature (1)..(10): P5-index
gcaagcctta

SEQ ID NO: 145 - DNA, 10 bp, Artificial Sequence
  Synthesied
  misc_feature (1)..(10): P5-index
ctgagtgtga

SEQ ID NO: 146 - DNA, 10 bp, Artificial Sequence
  Synthesied
  misc_feature (1)..(10): P5-index
agtcaccaac

SEQ ID NO: 147 - DNA, 10 bp, Artificial Sequence
  Synthesied
  misc_feature (1)..(10): P5-index
tactcaagcg

SEQ ID NO: 148 - DNA, 10 bp, Artificial Sequence
  Synthesied
  misc_feature (1)..(10): P5-index
gcagtgtctt

SEQ ID NO: 149 - DNA, 10 bp, Artificial Sequence
  Synthesied
  misc_feature (1)..(10): P5-index
catggtgcga

SEQ ID NO: 150 - DNA, 10 bp, Artificial Sequence
  Synthesied
  misc_feature (1)..(10): P5-index
ataacgcact

SEQ ID NO: 151 - DNA, 10 bp, Artificial Sequence
  Synthesied
  misc_feature (1)..(10): P5-index
ggctacatag

SEQ ID NO: 152 - DNA, 10 bp, Artificial Sequence
  Synthesied
  misc_feature (1)..(10): P5-index
tcgctatgtc

SEQ ID NO: 153 - DNA, 10 bp, Artificial Sequence
  Synthesied
  misc_feature (1)..(10): P5-index
cagtcatgtt

SEQ ID NO: 154 - DNA, 10 bp, Artificial Sequence
  Synthesied
  misc_feature (1)..(10): P5-index
atcagtatgg

SEQ ID NO: 155 - DNA, 10 bp, Artificial Sequence
  Synthesied
  misc_feature (1)..(10): P5-index
ggacaggcaa

SEQ ID NO: 156 - DNA, 10 bp, Artificial Sequence
  Synthesied
  misc_feature (1)..(10): P5-index
tctgtccacc

SEQ ID NO: 157 - DNA, 10 bp, Artificial Sequence
  Synthesied
  misc_feature (1)..(10): P5-index
agattccgcg

SEQ ID NO: 158 - DNA, 10 bp, Artificial Sequence
  Synthesied
  misc_feature (1)..(10): P5-index
caccgaataa

SEQ ID NO: 159 - DNA, 10 bp, Artificial Sequence
  Synthesied
  misc_feature (1)..(10): P5-index
ttgaagtctc

SEQ ID NO: 160 - DNA, 10 bp, Artificial Sequence
  Synthesied
  misc_feature (1)..(10): P5-index
gctgctgagt

SEQ ID NO: 161 - DNA, 10 bp, Artificial Sequence
  Synthesied
  misc_feature (1)..(10): P5-index
gacgctaacg

SEQ ID NO: 162 - DNA, 10 bp, Artificial Sequence
  Synthesied
  misc_feature (1)..(10): P5-index
ccacaattac

SEQ ID NO: 163 - DNA, 10 bp, Artificial Sequence
  Synthesied
  misc_feature (1)..(10): P5-index
attagccgtt

SEQ ID NO: 164 - DNA, 10 bp, Artificial Sequence
  Synthesied
  misc_feature (1)..(10): P5-index
tggttggcga

SEQ ID NO: 165 - DNA, 10 bp, Artificial Sequence
  Synthesied
  misc_feature (1)..(10): P5-index
gatggcgctt

SEQ ID NO: 166 - DNA, 10 bp, Artificial Sequence
  Synthesied
  misc_feature (1)..(10): P5-index
ctacaacaag

SEQ ID NO: 167 - DNA, 10 bp, Artificial Sequence
  Synthesied
  misc_feature (1)..(10): P5-index
aggattagga

SEQ ID NO: 168 - DNA, 10 bp, Artificial Sequence
  Synthesied
  misc_feature (1)..(10): P5-index
tcctcgttcc

SEQ ID NO: 169 - DNA, 10 bp, Artificial Sequence
  Synthesied
  misc_feature (1)..(10): P5-index
actcggactg

SEQ ID NO: 170 - DNA, 10 bp, Artificial Sequence
  Synthesied
  misc_feature (1)..(10): P5-index
gagaatctca

SEQ ID NO: 171 - DNA, 10 bp, Artificial Sequence
  Synthesied
  misc_feature (1)..(10): P5-index
ttcttctgac

SEQ ID NO: 172 - DNA, 10 bp, Artificial Sequence
  Synthesied
  misc_feature (1)..(10): P5-index
cgagcagagt

SEQ ID NO: 173 - DNA, 10 bp, Artificial Sequence
  Synthesied
  misc_feature (1)..(10): P5-index
cagacaaggt

SEQ ID NO: 174 - DNA, 10 bp, Artificial Sequence
  Synthesied
  misc_feature (1)..(10): P5-index
gctcacgaag

SEQ ID NO: 175 - DNA, 10 bp, Artificial Sequence
  Synthesied
  misc_feature (1)..(10): P5-index
ataggttctc

SEQ ID NO: 176 - DNA, 10 bp, Artificial Sequence
  Synthesied
  misc_feature (1)..(10): P5-index
tgcttgctca

SEQ ID NO: 177 - DNA, 10 bp, Artificial Sequence
  Synthesied
  misc_feature (1)..(10): P5-index
ttatctctcc

SEQ ID NO: 178 - DNA, 10 bp, Artificial Sequence
  Synthesied
  misc_feature (1)..(10): P5-index
gctggcaaga

SEQ ID NO: 179 - DNA, 10 bp, Artificial Sequence
  Synthesied
  misc_feature (1)..(10): P5-index
cagaagtgat

SEQ ID NO: 180 - DNA, 10 bp, Artificial Sequence
  Synthesied
  misc_feature (1)..(10): P5-index
agcctagctg

SEQ ID NO: 181 - DNA, 10 bp, Artificial Sequence
  Synthesied
  misc_feature (1)..(10): P5-index
acggaccgat

SEQ ID NO: 182 - DNA, 10 bp, Artificial Sequence
  Synthesied
  misc_feature (1)..(10): P5-index
ggcttggtta

SEQ ID NO: 183 - DNA, 10 bp, Artificial Sequence
  Synthesied
  misc_feature (1)..(10): P5-index
taacgaacgg

SEQ ID NO: 184 - DNA, 10 bp, Artificial Sequence
  Synthesied
  misc_feature (1)..(10): P5-index
cttacttacc

SEQ ID NO: 185 - DNA, 10 bp, Artificial Sequence
  Synthesied
  misc_feature (1)..(10): P5-index
ggccaaggta

SEQ ID NO: 186 - DNA, 10 bp, Artificial Sequence
  Synthesied
  misc_feature (1)..(10): P5-index
taagcgtcag

SEQ ID NO: 187 - DNA, 10 bp, Artificial Sequence
  Synthesied
  misc_feature (1)..(10): P5-index
actattcagc

SEQ ID NO: 188 - DNA, 10 bp, Artificial Sequence
  Synthesied
  misc_feature (1)..(10): P5-index
ctgtgcatct

SEQ ID NO: 189 - DNA, 10 bp, Artificial Sequence
  Synthesied
  misc_feature (1)..(10): P5-index
acggtatagc

SEQ ID NO: 190 - DNA, 10 bp, Artificial Sequence
  Synthesied
  misc_feature (1)..(10): P5-index
taatgcgcct

SEQ ID NO: 191 - DNA, 10 bp, Artificial Sequence
  Synthesied
  misc_feature (1)..(10): P5-index
cgtcctataa

SEQ ID NO: 192 - DNA, 10 bp, Artificial Sequence
  Synthesied
  misc_feature (1)..(10): P5-index
gtcaagcgtg

SEQ ID NO: 193 - DNA, 10 bp, Artificial Sequence
  Synthesied
  misc_feature (1)..(10): P5-index
ccaactgcct

SEQ ID NO: 194 - DNA, 10 bp, Artificial Sequence
  Synthesied
  misc_feature (1)..(10): P5-index
tattgacggc

SEQ ID NO: 195 - DNA, 10 bp, Artificial Sequence
  Synthesied
  misc_feature (1)..(10): P5-index
gtggagatta

SEQ ID NO: 196 - DNA, 10 bp, Artificial Sequence
  Synthesied
  misc_feature (1)..(10): P5-index
agcctctaag

SEQ ID NO: 197 - DNA, 10 bp, Artificial Sequence
  Synthesied
  misc_feature (1)..(10): P5-index
ccgccacaat

SEQ ID NO: 198 - DNA, 10 bp, Artificial Sequence
  Synthesied
  misc_feature (1)..(10): P5-index
aacaacacga

SEQ ID NO: 199 - DNA, 10 bp, Artificial Sequence
  Synthesied
  misc_feature (1)..(10): P5-index
gtattgtgtc

SEQ ID NO: 200 - DNA, 10 bp, Artificial Sequence
  Synthesied
  misc_feature (1)..(10): P5-index
tgtggtgtcg

SEQ ID NO: 201 - DNA, 10 bp, Artificial Sequence
  Synthesied
  misc_feature (1)..(10): P5-index
ctgccatgca

SEQ ID NO: 202 - DNA, 10 bp, Artificial Sequence
  Synthesied
  misc_feature (1)..(10): P5-index
aacaaggcac

SEQ ID NO: 203 - DNA, 10 bp, Artificial Sequence
  Synthesied
  misc_feature (1)..(10): P5-index
ggattcatgt

SEQ ID NO: 204 - DNA, 10 bp, Artificial Sequence
  Synthesied
  misc_feature (1)..(10): P5-index
tctggtcatg

SEQ ID NO: 205 - DNA, 10 bp, Artificial Sequence
  Synthesied
  misc_feature (1)..(10): P5-index
ccacagtcga

SEQ ID NO: 206 - DNA, 10 bp, Artificial Sequence
  Synthesied
  misc_feature (1)..(10): P5-index
aacagcgacc

SEQ ID NO: 207 - DNA, 10 bp, Artificial Sequence
  Synthesied
  misc_feature (1)..(10): P5-index
ttgtcacttg

SEQ ID NO: 208 - DNA, 10 bp, Artificial Sequence
  Synthesied
  misc_feature (1)..(10): P5-index
ggtgttagat

SEQ ID NO: 209 - DNA, 10 bp, Artificial Sequence
  Synthesied
  misc_feature (1)..(10): P5-index
ctggtaacgc

SEQ ID NO: 210 - DNA, 10 bp, Artificial Sequence
  Synthesied
  misc_feature (1)..(10): P5-index
aacagttgcg

SEQ ID NO: 211 - DNA, 10 bp, Artificial Sequence
  Synthesied
  misc_feature (1)..(10): P5-index
tgatcggaat

SEQ ID NO: 212 - DNA, 10 bp, Artificial Sequence
  Synthesied
  misc_feature (1)..(10): P5-index
gctcacctta

SEQ ID NO: 213 - DNA, 10 bp, Artificial Sequence
  Synthesied
  misc_feature (1)..(10): P5-index
ccgcactgaa

SEQ ID NO: 214 - DNA, 10 bp, Artificial Sequence
  Synthesied
  misc_feature (1)..(10): P5-index
aacatgatcc

SEQ ID NO: 215 - DNA, 10 bp, Artificial Sequence
  Synthesied
  misc_feature (1)..(10): P5-index
gtatgagctt

SEQ ID NO: 216 - DNA, 10 bp, Artificial Sequence
  Synthesied
  misc_feature (1)..(10): P5-index
tgtgctcagg

SEQ ID NO: 217 - DNA, 10 bp, Artificial Sequence
  Synthesied
  misc_feature (1)..(10): P5-index
ctaggtagcc

SEQ ID NO: 218 - DNA, 10 bp, Artificial Sequence
  Synthesied
  misc_feature (1)..(10): P5-index
aaccactcgg

SEQ ID NO: 219 - DNA, 10 bp, Artificial Sequence
  Synthesied
  misc_feature (1)..(10): P5-index
tgtacggata

SEQ ID NO: 220 - DNA, 10 bp, Artificial Sequence
  Synthesied
  misc_feature (1)..(10): P5-index
gcgttactat

SEQ ID NO: 221 - DNA, 10 bp, Artificial Sequence
  Synthesied
  misc_feature (1)..(10): P5-index
ccattgttgt

SEQ ID NO: 222 - DNA, 10 bp, Artificial Sequence
  Synthesied
  misc_feature (1)..(10): P5-index
aaccgaggac

SEQ ID NO: 223 - DNA, 10 bp, Artificial Sequence
  Synthesied
  misc_feature (1)..(10): P5-index
ggtactacca

SEQ ID NO: 224 - DNA, 10 bp, Artificial Sequence
  Synthesied
  misc_feature (1)..(10): P5-index
ttggaccatg

SEQ ID NO: 225 - DNA, 10 bp, Artificial Sequence
  Synthesied
  misc_feature (1)..(10): P5-index
cgagtggtat

SEQ ID NO: 226 - DNA, 10 bp, Artificial Sequence
  Synthesied
  misc_feature (1)..(10): P5-index
aagaccacgg

SEQ ID NO: 227 - DNA, 10 bp, Artificial Sequence
  Synthesied
  misc_feature (1)..(10): P5-index
tcttgacaca

SEQ ID NO: 228 - DNA, 10 bp, Artificial Sequence
  Synthesied
  misc_feature (1)..(10): P5-index
gtccattgtc

SEQ ID NO: 229 - DNA, 10 bp, Artificial Sequence
  Synthesied
  misc_feature (1)..(10): P5-index
cttcctccga

SEQ ID NO: 230 - DNA, 10 bp, Artificial Sequence
  Synthesied
  misc_feature (1)..(10): P5-index
aagaggaacg

SEQ ID NO: 231 - DNA, 10 bp, Artificial Sequence
  Synthesied
  misc_feature (1)..(10): P5-index
tcctaaggtt

SEQ ID NO: 232 - DNA, 10 bp, Artificial Sequence
  Synthesied
  misc_feature (1)..(10): P5-index
ggagtcttac

SEQ ID NO: 233 - DNA, 10 bp, Artificial Sequence
  Synthesied
  misc_feature (1)..(10): P5-index
ggaggtatga

SEQ ID NO: 234 - DNA, 10 bp, Artificial Sequence
  Synthesied
  misc_feature (1)..(10): P5-index
aagccgtaat

SEQ ID NO: 235 - DNA, 10 bp, Artificial Sequence
  Synthesied
  misc_feature (1)..(10): P5-index
tctaacggcc

SEQ ID NO: 236 - DNA, 10 bp, Artificial Sequence
  Synthesied
  misc_feature (1)..(10): P5-index
ctcttacctg

SEQ ID NO: 237 - DNA, 10 bp, Artificial Sequence
  Synthesied
  misc_feature (1)..(10): P5-index
cttgctaaca

SEQ ID NO: 238 - DNA, 10 bp, Artificial Sequence
  Synthesied
  misc_feature (1)..(10): P5-index
aagcggttac

SEQ ID NO: 239 - DNA, 10 bp, Artificial Sequence
  Synthesied
  misc_feature (1)..(10): P5-index
ggatacggtt

SEQ ID NO: 240 - DNA, 10 bp, Artificial Sequence
  Synthesied
  misc_feature (1)..(10): P5-index
tccataccgg

SEQ ID NO: 241 - DNA, 10 bp, Artificial Sequence
  Synthesied
  misc_feature (1)..(10): P5-index
ccatctggtt

SEQ ID NO: 242 - DNA, 10 bp, Artificial Sequence
  Synthesied
  misc_feature (1)..(10): P5-index
aagctgaaga

SEQ ID NO: 243 - DNA, 10 bp, Artificial Sequence
  Synthesied
  misc_feature (1)..(10): P5-index
ttcaactccg

SEQ ID NO: 244 - DNA, 10 bp, Artificial Sequence
  Synthesied
  misc_feature (1)..(10): P5-index
ggtggactac

SEQ ID NO: 245 - DNA, 10 bp, Artificial Sequence
  Synthesied
  misc_feature (1)..(10): P5-index
cgcatacttc

SEQ ID NO: 246 - DNA, 10 bp, Artificial Sequence
  Synthesied
  misc_feature (1)..(10): P5-index
aatcgcagca

SEQ ID NO: 247 - DNA, 10 bp, Artificial Sequence
  Synthesied
  misc_feature (1)..(10): P5-index
ttagagtcgg

SEQ ID NO: 248 - DNA, 10 bp, Artificial Sequence
  Synthesied
  misc_feature (1)..(10): P5-index
gcgtctgaat

SEQ ID NO: 249 - DNA, 10 bp, Artificial Sequence
  Synthesied
  misc_feature (1)..(10): P5-index
ctcctcatgt

SEQ ID NO: 250 - DNA, 10 bp, Artificial Sequence
  Synthesied
  misc_feature (1)..(10): P5-index
aattggccac

SEQ ID NO: 251 - DNA, 10 bp, Artificial Sequence
  Synthesied
  misc_feature (1)..(10): P5-index
tgaacatgtg

SEQ ID NO: 252 - DNA, 10 bp, Artificial Sequence
  Synthesied
  misc_feature (1)..(10): P5-index
gcggatgaca

SEQ ID NO: 253 - DNA, 10 bp, Artificial Sequence
  Synthesied
  misc_feature (1)..(10): P5-index
tggtgtaggc

SEQ ID NO: 254 - DNA, 10 bp, Artificial Sequence
  Synthesied
  misc_feature (1)..(10): P5-index
acaacagtct

SEQ ID NO: 255 - DNA, 10 bp, Artificial Sequence
  Synthesied
  misc_feature (1)..(10): P5-index
ctcgagtcta

SEQ ID NO: 256 - DNA, 10 bp, Artificial Sequence
  Synthesied
  misc_feature (1)..(10): P5-index
gatctccaag

SEQ ID NO: 257 - DNA, 10 bp, Artificial Sequence
  Synthesied
  misc_feature (1)..(10): P5-index
tgccgatacc

SEQ ID NO: 258 - DNA, 10 bp, Artificial Sequence
  Synthesied
  misc_feature (1)..(10): P5-index
acaatggttg

SEQ ID NO: 259 - DNA, 10 bp, Artificial Sequence
  Synthesied
  misc_feature (1)..(10): P5-index
cattacaggt

SEQ ID NO: 260 - DNA, 10 bp, Artificial Sequence
  Synthesied
  misc_feature (1)..(10): P5-index
gtggctccaa

SEQ ID NO: 261 - DNA, 10 bp, Artificial Sequence
  Synthesied
  misc_feature (1)..(10): P5-index
gtcgaggttc

SEQ ID NO: 262 - DNA, 10 bp, Artificial Sequence
  Synthesied
  misc_feature (1)..(10): P5-index
acacgcaagt

SEQ ID NO: 263 - DNA, 10 bp, Artificial Sequence
  Synthesied
  misc_feature (1)..(10): P5-index
cgttcttgca

SEQ ID NO: 264 - DNA, 10 bp, Artificial Sequence
  Synthesied
  misc_feature (1)..(10): P5-index
tagataccag

SEQ ID NO: 265 - DNA, 10 bp, Artificial Sequence
  Synthesied
  misc_feature (1)..(10): P5-index
gagctcagac

SEQ ID NO: 266 - DNA, 10 bp, Artificial Sequence
  Synthesied
  misc_feature (1)..(10): P5-index
accaattctg

SEQ ID NO: 267 - DNA, 10 bp, Artificial Sequence
  Synthesied
  misc_feature (1)..(10): P5-index
tgttgagaga

SEQ ID NO: 268 - DNA, 10 bp, Artificial Sequence
  Synthesied
  misc_feature (1)..(10): P5-index
ctagcgctct

SEQ ID NO: 269 - DNA, 10 bp, Artificial Sequence
  Synthesied
  misc_feature (1)..(10): P5-index
tgagttacag

SEQ ID NO: 270 - DNA, 10 bp, Artificial Sequence
  Synthesied
  misc_feature (1)..(10): P5-index
accacactcc

SEQ ID NO: 271 - DNA, 10 bp, Artificial Sequence
  Synthesied
  misc_feature (1)..(10): P5-index
gattggtaga

SEQ ID NO: 272 - DNA, 10 bp, Artificial Sequence
  Synthesied
  misc_feature (1)..(10): P5-index
ctgcacggtt

SEQ ID NO: 273 - DNA, 10 bp, Artificial Sequence
  Synthesied
  misc_feature (1)..(10): P5-index
tgtcgatcat

SEQ ID NO: 274 - DNA, 10 bp, Artificial Sequence
  Synthesied
  misc_feature (1)..(10): P5-index
acgaagctcg

SEQ ID NO: 275 - DNA, 10 bp, Artificial Sequence
  Synthesied
  misc_feature (1)..(10): P5-index
cacttcgata

SEQ ID NO: 276 - DNA, 10 bp, Artificial Sequence
  Synthesied
  misc_feature (1)..(10): P5-index
gtagctaggc

SEQ ID NO: 277 - DNA, 10 bp, Artificial Sequence
  Synthesied
  misc_feature (1)..(10): P5-index
cagttccgta

SEQ ID NO: 278 - DNA, 10 bp, Artificial Sequence
  Synthesied
  misc_feature (1)..(10): P5-index
agcgcattgt

SEQ ID NO: 279 - DNA, 10 bp, Artificial Sequence
  Synthesied
  misc_feature (1)..(10): P5-index
ttacagaacc

SEQ ID NO: 280 - DNA, 10 bp, Artificial Sequence
  Synthesied
  misc_feature (1)..(10): P5-index
gctagtgcag

SEQ ID NO: 281 - DNA, 10 bp, Artificial Sequence
  Synthesied
  misc_feature (1)..(10): P5-index
tacgtatcac

SEQ ID NO: 282 - DNA, 10 bp, Artificial Sequence
  Synthesied
  misc_feature (1)..(10): P5-index
aggagcgttg

SEQ ID NO: 283 - DNA, 10 bp, Artificial Sequence
  Synthesied
  misc_feature (1)..(10): P5-index
gtatctcact

SEQ ID NO: 284 - DNA, 10 bp, Artificial Sequence
  Synthesied
  misc_feature (1)..(10): P5-index
cctcagagga

SEQ ID NO: 285 - DNA, 10 bp, Artificial Sequence
  Synthesied
  misc_feature (1)..(10): P5-index
ggcactccta

SEQ ID NO: 286 - DNA, 10 bp, Artificial Sequence
  Synthesied
  misc_feature (1)..(10): P5-index
caacagaagt

SEQ ID NO: 287 - DNA, 10 bp, Artificial Sequence
  Synthesied
  misc_feature (1)..(10): P5-index
attgtcttcg

SEQ ID NO: 288 - DNA, 10 bp, Artificial Sequence
  Synthesied
  misc_feature (1)..(10): P5-index
tcgtgaggac

SEQ ID NO: 289 - DNA, 10 bp, Artificial Sequence
  Synthesied
  misc_feature (1)..(10): P5-index
gtcagcatct

SEQ ID NO: 290 - DNA, 10 bp, Artificial Sequence
  Synthesied
  misc_feature (1)..(10): P5-index
caaccatgta

SEQ ID NO: 291 - DNA, 10 bp, Artificial Sequence
  Synthesied
  misc_feature (1)..(10): P5-index
agttaggcgg

SEQ ID NO: 292 - DNA, 10 bp, Artificial Sequence
  Synthesied
  misc_feature (1)..(10): P5-index
tcggttcaac

SEQ ID NO: 293 - DNA, 10 bp, Artificial Sequence
  Synthesied
  misc_feature (1)..(10): P5-index
gttagtcgat

SEQ ID NO: 294 - DNA, 10 bp, Artificial Sequence
  Synthesied
  misc_feature (1)..(10): P5-index
caattcgcgg

SEQ ID NO: 295 - DNA, 10 bp, Artificial Sequence
  Synthesied
  misc_feature (1)..(10): P5-index
aggcaatacc

SEQ ID NO: 296 - DNA, 10 bp, Artificial Sequence
  Synthesied
  misc_feature (1)..(10): P5-index
tccgcgatta

SEQ ID NO: 297 - DNA, 10 bp, Artificial Sequence
  Synthesied
  misc_feature (1)..(10): P5-index
gctgtacgag

SEQ ID NO: 298 - DNA, 10 bp, Artificial Sequence
  Synthesied
  misc_feature (1)..(10): P5-index
cagagtaacc

SEQ ID NO: 299 - DNA, 10 bp, Artificial Sequence
  Synthesied
  misc_feature (1)..(10): P5-index
ttaccgtcta

SEQ ID NO: 300 - DNA, 10 bp, Artificial Sequence
  Synthesied
  misc_feature (1)..(10): P5-index
agctacgtgt

SEQ ID NO: 301 - DNA, 10 bp, Artificial Sequence
  Synthesied
  misc_feature (1)..(10): P5-index
gtcactggta

SEQ ID NO: 302 - DNA, 10 bp, Artificial Sequence
  Synthesied
  misc_feature (1)..(10): P5-index
catgtcacat

SEQ ID NO: 303 - DNA, 10 bp, Artificial Sequence
  Synthesied
  misc_feature (1)..(10): P5-index
agatggtacc

SEQ ID NO: 304 - DNA, 10 bp, Artificial Sequence
  Synthesied
  misc_feature (1)..(10): P5-index
tcgcaactgg

SEQ ID NO: 305 - DNA, 10 bp, Artificial Sequence
  Synthesied
  misc_feature (1)..(10): P5-index
tcaaccttgg

SEQ ID NO: 306 - DNA, 10 bp, Artificial Sequence
  Synthesied
  misc_feature (1)..(10): P5-index
cattgagacc

SEQ ID NO: 307 - DNA, 10 bp, Artificial Sequence
  Synthesied
  misc_feature (1)..(10): P5-index
aggcatcgaa

SEQ ID NO: 308 - DNA, 10 bp, Artificial Sequence
  Synthesied
  misc_feature (1)..(10): P5-index
gtcgtgactt

SEQ ID NO: 309 - DNA, 10 bp, Artificial Sequence
  Synthesied
  misc_feature (1)..(10): P5-index
agtgtaccgc

SEQ ID NO: 310 - DNA, 10 bp, Artificial Sequence
  Synthesied
  misc_feature (1)..(10): P5-index
ccatgtatct

SEQ ID NO: 311 - DNA, 10 bp, Artificial Sequence
  Synthesied
  misc_feature (1)..(10): P5-index
tagacgtatg

SEQ ID NO: 312 - DNA, 10 bp, Artificial Sequence
  Synthesied
  misc_feature (1)..(10): P5-index
gtccacggaa

SEQ ID NO: 313 - DNA, 10 bp, Artificial Sequence
  Synthesied
  misc_feature (1)..(10): P5-index
ggctcctcaa

SEQ ID NO: 314 - DNA, 10 bp, Artificial Sequence
  Synthesied
  misc_feature (1)..(10): P5-index
ccgaatagtt

SEQ ID NO: 315 - DNA, 10 bp, Artificial Sequence
  Synthesied
  misc_feature (1)..(10): P5-index
aatgtagagg

SEQ ID NO: 316 - DNA, 10 bp, Artificial Sequence
  Synthesied
  misc_feature (1)..(10): P5-index
ttacggctcc

SEQ ID NO: 317 - DNA, 10 bp, Artificial Sequence
  Synthesied
  misc_feature (1)..(10): P5-index
tacctcacag

SEQ ID NO: 318 - DNA, 10 bp, Artificial Sequence
  Synthesied
  misc_feature (1)..(10): P5-index
cctagttggt

SEQ ID NO: 319 - DNA, 10 bp, Artificial Sequence
  Synthesied
  misc_feature (1)..(10): P5-index
ggagaagata

SEQ ID NO: 320 - DNA, 10 bp, Artificial Sequence
  Synthesied
  misc_feature (1)..(10): P5-index
atgtcgctcc

SEQ ID NO: 321 - DNA, 10 bp, Artificial Sequence
  Synthesied
  misc_feature (1)..(10): P5-index
agactcagga

SEQ ID NO: 322 - DNA, 10 bp, Artificial Sequence
  Synthesied
  misc_feature (1)..(10): P5-index
cctgcatatc

SEQ ID NO: 323 - DNA, 10 bp, Artificial Sequence
  Synthesied
  misc_feature (1)..(10): P5-index
tagaaggcct

SEQ ID NO: 324 - DNA, 10 bp, Artificial Sequence
  Synthesied
  misc_feature (1)..(10): P5-index
gtctgtctag

SEQ ID NO: 325 - DNA, 10 bp, Artificial Sequence
  Synthesied
  misc_feature (1)..(10): P5-index
aggagtgcac

SEQ ID NO: 326 - DNA, 10 bp, Artificial Sequence
  Synthesied
  misc_feature (1)..(10): P5-index
ccttcaagta

SEQ ID NO: 327 - DNA, 10 bp, Artificial Sequence
  Synthesied
  misc_feature (1)..(10): P5-index
tacgagtagt

SEQ ID NO: 328 - DNA, 10 bp, Artificial Sequence
  Synthesied
  misc_feature (1)..(10): P5-index
gtactcctcg

SEQ ID NO: 329 - DNA, 10 bp, Artificial Sequence
  Synthesied
  misc_feature (1)..(10): P5-index
gaccacaagg

SEQ ID NO: 330 - DNA, 10 bp, Artificial Sequence
  Synthesied
  misc_feature (1)..(10): P5-index
cgttgattcc

SEQ ID NO: 331 - DNA, 10 bp, Artificial Sequence
  Synthesied
  misc_feature (1)..(10): P5-index
atagtggcaa

SEQ ID NO: 332 - DNA, 10 bp, Artificial Sequence
  Synthesied
  misc_feature (1)..(10): P5-index
tcgactcgtt

SEQ ID NO: 333 - DNA, 10 bp, Artificial Sequence
  Synthesied
  misc_feature (1)..(10): P5-index
tagcagccag

SEQ ID NO: 334 - DNA, 10 bp, Artificial Sequence
  Synthesied
  misc_feature (1)..(10): P5-index
ctaggaattc

SEQ ID NO: 335 - DNA, 10 bp, Artificial Sequence
  Synthesied
  misc_feature (1)..(10): P5-index
agtattggct

SEQ ID NO: 336 - DNA, 10 bp, Artificial Sequence
  Synthesied
  misc_feature (1)..(10): P5-index
gcctcctaga

SEQ ID NO: 337 - DNA, 10 bp, Artificial Sequence
  Synthesied
  misc_feature (1)..(10): P5-index
agacgactgc

SEQ ID NO: 338 - DNA, 10 bp, Artificial Sequence
  Synthesied
  misc_feature (1)..(10): P5-index
ctcaatgact

SEQ ID NO: 339 - DNA, 10 bp, Artificial Sequence
  Synthesied
  misc_feature (1)..(10): P5-index
tcttcgagaa

SEQ ID NO: 340 - DNA, 10 bp, Artificial Sequence
  Synthesied
  misc_feature (1)..(10): P5-index
gaggtctctg

SEQ ID NO: 341 - DNA, 10 bp, Artificial Sequence
  Synthesied
  misc_feature (1)..(10): P5-index
atgcttggag

SEQ ID NO: 342 - DNA, 10 bp, Artificial Sequence
  Synthesied
  misc_feature (1)..(10): P5-index
ggatacctcc

SEQ ID NO: 343 - DNA, 10 bp, Artificial Sequence
  Synthesied
  misc_feature (1)..(10): P5-index
catgcaacta

SEQ ID NO: 344 - DNA, 10 bp, Artificial Sequence
  Synthesied
  misc_feature (1)..(10): P5-index
tccaggtagt

SEQ ID NO: 345 - DNA, 10 bp, Artificial Sequence
  Synthesied
  misc_feature (1)..(10): P5-index
ggttgcagta

SEQ ID NO: 346 - DNA, 10 bp, Artificial Sequence
  Synthesied
  misc_feature (1)..(10): P5-index
tcagaagcac

SEQ ID NO: 347 - DNA, 10 bp, Artificial Sequence
  Synthesied
  misc_feature (1)..(10): P5-index
atgcttctgt

SEQ ID NO: 348 - DNA, 10 bp, Artificial Sequence
  Synthesied
  misc_feature (1)..(10): P5-index
cacacgtacg

SEQ ID NO: 349 - DNA, 10 bp, Artificial Sequence
  Synthesied
  misc_feature (1)..(10): P5-index
ctctaggcca

SEQ ID NO: 350 - DNA, 10 bp, Artificial Sequence
  Synthesied
  misc_feature (1)..(10): P5-index
acaatcctag

SEQ ID NO: 351 - DNA, 10 bp, Artificial Sequence
  Synthesied
  misc_feature (1)..(10): P5-index
ggtggaagtt

SEQ ID NO: 352 - DNA, 10 bp, Artificial Sequence
  Synthesied
  misc_feature (1)..(10): P5-index
tagccttagc

SEQ ID NO: 353 - DNA, 10 bp, Artificial Sequence
  Synthesied
  misc_feature (1)..(10): P5-index
tggactcaca

SEQ ID NO: 354 - DNA, 10 bp, Artificial Sequence
  Synthesied
  misc_feature (1)..(10): P5-index
acctaagtgc

SEQ ID NO: 355 - DNA, 10 bp, Artificial Sequence
  Synthesied
  misc_feature (1)..(10): P5-index
gaactgagtg

SEQ ID NO: 356 - DNA, 10 bp, Artificial Sequence
  Synthesied
  misc_feature (1)..(10): P5-index
cttggctcat

SEQ ID NO: 357 - DNA, 10 bp, Artificial Sequence
  Synthesied
  misc_feature (1)..(10): P5-index
gttcgaacct

SEQ ID NO: 358 - DNA, 10 bp, Artificial Sequence
  Synthesied
  misc_feature (1)..(10): P5-index
acgacttaac

SEQ ID NO: 359 - DNA, 10 bp, Artificial Sequence
  Synthesied
  misc_feature (1)..(10): P5-index
tgagacggta

SEQ ID NO: 360 - DNA, 10 bp, Artificial Sequence
  Synthesied
  misc_feature (1)..(10): P5-index
cacttgctgg

SEQ ID NO: 361 - DNA, 10 bp, Artificial Sequence
  Synthesied
  misc_feature (1)..(10): P5-index
catgcctagt

SEQ ID NO: 362 - DNA, 10 bp, Artificial Sequence
  Synthesied
  misc_feature (1)..(10): P5-index
atacatggcc

SEQ ID NO: 363 - DNA, 10 bp, Artificial Sequence
  Synthesied
  misc_feature (1)..(10): P5-index
tggatacttg

SEQ ID NO: 364 - DNA, 10 bp, Artificial Sequence
  Synthesied
  misc_feature (1)..(10): P5-index
gcctggacaa

SEQ ID NO: 365 - DNA, 10 bp, Artificial Sequence
  Synthesied
  misc_feature (1)..(10): P5-index
catctagtgg

SEQ ID NO: 366 - DNA, 10 bp, Artificial Sequence
  Synthesied
  misc_feature (1)..(10): P5-index
atagagcgat

SEQ ID NO: 367 - DNA, 10 bp, Artificial Sequence
  Synthesied
  misc_feature (1)..(10): P5-index
ggcagcaaca

SEQ ID NO: 368 - DNA, 10 bp, Artificial Sequence
  Synthesied
  misc_feature (1)..(10): P5-index
tcgtcttctc

SEQ ID NO: 369 - DNA, 10 bp, Artificial Sequence
  Synthesied
  misc_feature (1)..(10): P5-index
gaacggccat

SEQ ID NO: 370 - DNA, 10 bp, Artificial Sequence
  Synthesied
  misc_feature (1)..(10): P5-index
attaacggtg

SEQ ID NO: 371 - DNA, 10 bp, Artificial Sequence
  Synthesied
  misc_feature (1)..(10): P5-index
cggttaatga

SEQ ID NO: 372 - DNA, 10 bp, Artificial Sequence
  Synthesied
  misc_feature (1)..(10): P5-index
tccgcttacc

SEQ ID NO: 373 - DNA, 10 bp, Artificial Sequence
  Synthesied
  misc_feature (1)..(10): P5-index
gcgtatcatt

SEQ ID NO: 374 - DNA, 10 bp, Artificial Sequence
  Synthesied
  misc_feature (1)..(10): P5-index
caaggcagac

SEQ ID NO: 375 - DNA, 10 bp, Artificial Sequence
  Synthesied
  misc_feature (1)..(10): P5-index
attctgttgg

SEQ ID NO: 376 - DNA, 10 bp, Artificial Sequence
  Synthesied
  misc_feature (1)..(10): P5-index
tgcacagcca

SEQ ID NO: 377 - DNA, 10 bp, Artificial Sequence
  Synthesied
  misc_feature (1)..(10): P5-index
tctcgcatcg

SEQ ID NO: 378 - DNA, 10 bp, Artificial Sequence
  Synthesied
  misc_feature (1)..(10): P5-index
caatcaccat

SEQ ID NO: 379 - DNA, 10 bp, Artificial Sequence
  Synthesied
  misc_feature (1)..(10): P5-index
gtgaatgaga

SEQ ID NO: 380 - DNA, 10 bp, Artificial Sequence
  Synthesied
  misc_feature (1)..(10): P5-index
agcgtgtgtc

SEQ ID NO: 381 - DNA, 10 bp, Artificial Sequence
  Synthesied
  misc_feature (1)..(10): P5-index
gcaccttcat

SEQ ID NO: 382 - DNA, 10 bp, Artificial Sequence
  Synthesied
  misc_feature (1)..(10): P5-index
cgcttacaga

SEQ ID NO: 383 - DNA, 10 bp, Artificial Sequence
  Synthesied
  misc_feature (1)..(10): P5-index
tataggagtc

SEQ ID NO: 384 - DNA, 10 bp, Artificial Sequence
  Synthesied
  misc_feature (1)..(10): P5-index
atggacgtcg

SEQ ID NO: 385 - DNA, 10 bp, Artificial Sequence
  Synthesied
  misc_feature (1)..(10): P5-index
tctgtgcgta

SEQ ID NO: 386 - DNA, 10 bp, Artificial Sequence
  Synthesied
  misc_feature (1)..(10): P5-index
gaacattcct

SEQ ID NO: 387 - DNA, 10 bp, Artificial Sequence
  Synthesied
  misc_feature (1)..(10): P5-index
ctgagagaag

SEQ ID NO: 388 - DNA, 10 bp, Artificial Sequence
  Synthesied
  misc_feature (1)..(10): P5-index
agctccatgc

SEQ ID NO: 389 - DNA, 10 bp, Artificial Sequence
  Synthesied
  misc_feature (1)..(10): P5-index
atacctgcga

SEQ ID NO: 390 - DNA, 10 bp, Artificial Sequence
  Synthesied
  misc_feature (1)..(10): P5-index
gccgaattag

SEQ ID NO: 391 - DNA, 10 bp, Artificial Sequence
  Synthesied
  misc_feature (1)..(10): P5-index
tatagccatc

SEQ ID NO: 392 - DNA, 10 bp, Artificial Sequence
  Synthesied
  misc_feature (1)..(10): P5-index
cggttgagct

SEQ ID NO: 393 - DNA, 10 bp, Artificial Sequence
  Synthesied
  misc_feature (1)..(10): P5-index
ctacatccac

SEQ ID NO: 394 - DNA, 10 bp, Artificial Sequence
  Synthesied
  misc_feature (1)..(10): P5-index
ggtataagtg

SEQ ID NO: 395 - DNA, 10 bp, Artificial Sequence
  Synthesied
  misc_feature (1)..(10): P5-index
tcgtcgtagt

SEQ ID NO: 396 - DNA, 10 bp, Artificial Sequence
  Synthesied
  misc_feature (1)..(10): P5-index
aacggcgtca

SEQ ID NO: 397 - DNA, 10 bp, Artificial Sequence
  Synthesied
  misc_feature (1)..(10): P5-index
tagtctgcta

SEQ ID NO: 398 - DNA, 10 bp, Artificial Sequence
  Synthesied
  misc_feature (1)..(10): P5-index
gtaagacacg

SEQ ID NO: 399 - DNA, 10 bp, Artificial Sequence
  Synthesied
  misc_feature (1)..(10): P5-index
cgcgagatat

SEQ ID NO: 400 - DNA, 10 bp, Artificial Sequence
  Synthesied
  misc_feature (1)..(10): P5-index
actctctggc

SEQ ID NO: 401 - DNA, 10 bp, Artificial Sequence
  Synthesied
  misc_feature (1)..(10): P5-index
gccatctcaa

SEQ ID NO: 402 - DNA, 10 bp, Artificial Sequence
  Synthesied
  misc_feature (1)..(10): P5-index
taaccacgcc

SEQ ID NO: 403 - DNA, 10 bp, Artificial Sequence
  Synthesied
  misc_feature (1)..(10): P5-index
cttgaggagt

SEQ ID NO: 404 - DNA, 10 bp, Artificial Sequence
  Synthesied
  misc_feature (1)..(10): P5-index
aggtgtattg

SEQ ID NO: 405 - DNA, 10 bp, Artificial Sequence
  Synthesied
  misc_feature (1)..(10): P5-index
atgccaggct

SEQ ID NO: 406 - DNA, 10 bp, Artificial Sequence
  Synthesied
  misc_feature (1)..(10): P5-index
tccttgaatc

SEQ ID NO: 407 - DNA, 10 bp, Artificial Sequence
  Synthesied
  misc_feature (1)..(10): P5-index
cgaagttcaa

SEQ ID NO: 408 - DNA, 10 bp, Artificial Sequence
  Synthesied
  misc_feature (1)..(10): P5-index
gatgacctgg

SEQ ID NO: 409 - DNA, 10 bp, Artificial Sequence
  Synthesied
  misc_feature (1)..(10): P5-index
agtgagttct

SEQ ID NO: 410 - DNA, 10 bp, Artificial Sequence
  Synthesied
  misc_feature (1)..(10): P5-index
tcgatagagc

SEQ ID NO: 411 - DNA, 10 bp, Artificial Sequence
  Synthesied
  misc_feature (1)..(10): P5-index
gaacgtcgaa

SEQ ID NO: 412 - DNA, 10 bp, Artificial Sequence
  Synthesied
  misc_feature (1)..(10): P5-index
ctctccactg

SEQ ID NO: 413 - DNA, 10 bp, Artificial Sequence
  Synthesied
  misc_feature (1)..(10): P5-index
gactagtaag

SEQ ID NO: 414 - DNA, 10 bp, Artificial Sequence
  Synthesied
  misc_feature (1)..(10): P5-index
tgacctactt

SEQ ID NO: 415 - DNA, 10 bp, Artificial Sequence
  Synthesied
  misc_feature (1)..(10): P5-index
cttgtcgtgc

SEQ ID NO: 416 - DNA, 10 bp, Artificial Sequence
  Synthesied
  misc_feature (1)..(10): P5-index
acgagacgca

SEQ ID NO: 417 - DNA, 10 bp, Artificial Sequence
  Synthesied
  misc_feature (1)..(10): P5-index
cgaaccgtac

SEQ ID NO: 418 - DNA, 10 bp, Artificial Sequence
  Synthesied
  misc_feature (1)..(10): P5-index
ttcctgagca

SEQ ID NO: 419 - DNA, 10 bp, Artificial Sequence
  Synthesied
  misc_feature (1)..(10): P5-index
aaggaacctt

SEQ ID NO: 420 - DNA, 10 bp, Artificial Sequence
  Synthesied
  misc_feature (1)..(10): P5-index
gcttgttagg

SEQ ID NO: 421 - DNA, 10 bp, Artificial Sequence
  Synthesied
  misc_feature (1)..(10): P7-index
aacgcgtcct

SEQ ID NO: 422 - DNA, 10 bp, Artificial Sequence
  Synthesied
  misc_feature (1)..(10): P7-index
ttaattcggc

SEQ ID NO: 423 - DNA, 10 bp, Artificial Sequence
  Synthesied
  misc_feature (1)..(10): P7-index
ggttaagaag

SEQ ID NO: 424 - DNA, 10 bp, Artificial Sequence
  Synthesied
  misc_feature (1)..(10): P7-index
ccgcgcatta

SEQ ID NO: 425 - DNA, 10 bp, Artificial Sequence
  Synthesied
  misc_feature (1)..(10): P7-index
tctcatggct

SEQ ID NO: 426 - DNA, 10 bp, Artificial Sequence
  Synthesied
  misc_feature (1)..(10): P7-index
gaattaacgg

SEQ ID NO: 427 - DNA, 10 bp, Artificial Sequence
  Synthesied
  misc_feature (1)..(10): P7-index
agcaggctac

SEQ ID NO: 428 - DNA, 10 bp, Artificial Sequence
  Synthesied
  misc_feature (1)..(10): P7-index
ctggcctata

SEQ ID NO: 429 - DNA, 10 bp, Artificial Sequence
  Synthesied
  misc_feature (1)..(10): P7-index
gcatctgatc

SEQ ID NO: 430 - DNA, 10 bp, Artificial Sequence
  Synthesied
  misc_feature (1)..(10): P7-index
tatgtcctgg

SEQ ID NO: 431 - DNA, 10 bp, Artificial Sequence
  Synthesied
  misc_feature (1)..(10): P7-index
ctgaagacaa

SEQ ID NO: 432 - DNA, 10 bp, Artificial Sequence
  Synthesied
  misc_feature (1)..(10): P7-index
agccgatgct

SEQ ID NO: 433 - DNA, 10 bp, Artificial Sequence
  Synthesied
  misc_feature (1)..(10): P7-index
gttgcctcat

SEQ ID NO: 434 - DNA, 10 bp, Artificial Sequence
  Synthesied
  misc_feature (1)..(10): P7-index
tgcaatggcc

SEQ ID NO: 435 - DNA, 10 bp, Artificial Sequence
  Synthesied
  misc_feature (1)..(10): P7-index
ccattacatg

SEQ ID NO: 436 - DNA, 10 bp, Artificial Sequence
  Synthesied
  misc_feature (1)..(10): P7-index
aagcggatga

SEQ ID NO: 437 - DNA, 10 bp, Artificial Sequence
  Synthesied
  misc_feature (1)..(10): P7-index
attggtggtt

SEQ ID NO: 438 - DNA, 10 bp, Artificial Sequence
  Synthesied
  misc_feature (1)..(10): P7-index
tggttactga

SEQ ID NO: 439 - DNA, 10 bp, Artificial Sequence
  Synthesied
  misc_feature (1)..(10): P7-index
gcaacgacac

SEQ ID NO: 440 - DNA, 10 bp, Artificial Sequence
  Synthesied
  misc_feature (1)..(10): P7-index
caccactacg

SEQ ID NO: 441 - DNA, 10 bp, Artificial Sequence
  Synthesied
  misc_feature (1)..(10): P7-index
tacgcttacg

SEQ ID NO: 442 - DNA, 10 bp, Artificial Sequence
  Synthesied
  misc_feature (1)..(10): P7-index
gcacaagtaa

SEQ ID NO: 443 - DNA, 10 bp, Artificial Sequence
  Synthesied
  misc_feature (1)..(10): P7-index
cttatcacgc

SEQ ID NO: 444 - DNA, 10 bp, Artificial Sequence
  Synthesied
  misc_feature (1)..(10): P7-index
aggtggcgtt

SEQ ID NO: 445 - DNA, 10 bp, Artificial Sequence
  Synthesied
  misc_feature (1)..(10): P7-index
cgtgccttca

SEQ ID NO: 446 - DNA, 10 bp, Artificial Sequence
  Synthesied
  misc_feature (1)..(10): P7-index
gtgtgaagat

SEQ ID NO: 447 - DNA, 10 bp, Artificial Sequence
  Synthesied
  misc_feature (1)..(10): P7-index
aacattgagc

SEQ ID NO: 448 - DNA, 10 bp, Artificial Sequence
  Synthesied
  misc_feature (1)..(10): P7-index
tcacagcctg

SEQ ID NO: 449 - DNA, 10 bp, Artificial Sequence
  Synthesied
  misc_feature (1)..(10): P7-index
gcttgtctaa

SEQ ID NO: 450 - DNA, 10 bp, Artificial Sequence
  Synthesied
  misc_feature (1)..(10): P7-index
cggatgactt

SEQ ID NO: 451 - DNA, 10 bp, Artificial Sequence
  Synthesied
  misc_feature (1)..(10): P7-index
aacgacgagg

SEQ ID NO: 452 - DNA, 10 bp, Artificial Sequence
  Synthesied
  misc_feature (1)..(10): P7-index
ttaccatgcc

SEQ ID NO: 453 - DNA, 10 bp, Artificial Sequence
  Synthesied
  misc_feature (1)..(10): P7-index
tactatctcc

SEQ ID NO: 454 - DNA, 10 bp, Artificial Sequence
  Synthesied
  misc_feature (1)..(10): P7-index
ccgctaagaa

SEQ ID NO: 455 - DNA, 10 bp, Artificial Sequence
  Synthesied
  misc_feature (1)..(10): P7-index
ggaggctagt

SEQ ID NO: 456 - DNA, 10 bp, Artificial Sequence
  Synthesied
  misc_feature (1)..(10): P7-index
attacggctg

SEQ ID NO: 457 - DNA, 10 bp, Artificial Sequence
  Synthesied
  misc_feature (1)..(10): P7-index
gctggtagac

SEQ ID NO: 458 - DNA, 10 bp, Artificial Sequence
  Synthesied
  misc_feature (1)..(10): P7-index
taactgttgg

SEQ ID NO: 459 - DNA, 10 bp, Artificial Sequence
  Synthesied
  misc_feature (1)..(10): P7-index
cggaacgcta

SEQ ID NO: 460 - DNA, 10 bp, Artificial Sequence
  Synthesied
  misc_feature (1)..(10): P7-index
atctcacact

SEQ ID NO: 461 - DNA, 10 bp, Artificial Sequence
  Synthesied
  misc_feature (1)..(10): P7-index
tcgttggtct

SEQ ID NO: 462 - DNA, 10 bp, Artificial Sequence
  Synthesied
  misc_feature (1)..(10): P7-index
ggtgctcaag

SEQ ID NO: 463 - DNA, 10 bp, Artificial Sequence
  Synthesied
  misc_feature (1)..(10): P7-index
caacaatcgc

SEQ ID NO: 464 - DNA, 10 bp, Artificial Sequence
  Synthesied
  misc_feature (1)..(10): P7-index
atcagcagta

SEQ ID NO: 465 - DNA, 10 bp, Artificial Sequence
  Synthesied
  misc_feature (1)..(10): P7-index
gttgttgatc

SEQ ID NO: 466 - DNA, 10 bp, Artificial Sequence
  Synthesied
  misc_feature (1)..(10): P7-index
acgaggctca

SEQ ID NO: 467 - DNA, 10 bp, Artificial Sequence
  Synthesied
  misc_feature (1)..(10): P7-index
caaccaacag

SEQ ID NO: 468 - DNA, 10 bp, Artificial Sequence
  Synthesied
  misc_feature (1)..(10): P7-index
tgctactggt

SEQ ID NO: 469 - DNA, 10 bp, Artificial Sequence
  Synthesied
  misc_feature (1)..(10): P7-index
tgctactggt

SEQ ID NO: 470 - DNA, 10 bp, Artificial Sequence
  Synthesied
  misc_feature (1)..(10): P7-index
tcgccaatgg

SEQ ID NO: 471 - DNA, 10 bp, Artificial Sequence
  Synthesied
  misc_feature (1)..(10): P7-index
aactagcctc

SEQ ID NO: 472 - DNA, 10 bp, Artificial Sequence
  Synthesied
  misc_feature (1)..(10): P7-index
gtaatcggat

SEQ ID NO: 473 - DNA, 10 bp, Artificial Sequence
  Synthesied
  misc_feature (1)..(10): P7-index
agccagcgat

SEQ ID NO: 474 - DNA, 10 bp, Artificial Sequence
  Synthesied
  misc_feature (1)..(10): P7-index
gcaagttcta

SEQ ID NO: 475 - DNA, 10 bp, Artificial Sequence
  Synthesied
  misc_feature (1)..(10): P7-index
cattcaatgg

SEQ ID NO: 476 - DNA, 10 bp, Artificial Sequence
  Synthesied
  misc_feature (1)..(10): P7-index
ttggtcgacc

SEQ ID NO: 477 - DNA, 10 bp, Artificial Sequence
  Synthesied
  misc_feature (1)..(10): P7-index
tgtcctctgc

SEQ ID NO: 478 - DNA, 10 bp, Artificial Sequence
  Synthesied
  misc_feature (1)..(10): P7-index
gaataggaca

SEQ ID NO: 479 - DNA, 10 bp, Artificial Sequence
  Synthesied
  misc_feature (1)..(10): P7-index
ctgatctgtt

SEQ ID NO: 480 - DNA, 10 bp, Artificial Sequence
  Synthesied
  misc_feature (1)..(10): P7-index
accggaacag

SEQ ID NO: 481 - DNA, 10 bp, Artificial Sequence
  Synthesied
  misc_feature (1)..(10): P7-index
agatagagga

SEQ ID NO: 482 - DNA, 10 bp, Artificial Sequence
  Synthesied
  misc_feature (1)..(10): P7-index
tcgactgcag

SEQ ID NO: 483 - DNA, 10 bp, Artificial Sequence
  Synthesied
  misc_feature (1)..(10): P7-index
gatgtcttct

SEQ ID NO: 484 - DNA, 10 bp, Artificial Sequence
  Synthesied
  misc_feature (1)..(10): P7-index
ctccgacatc

SEQ ID NO: 485 - DNA, 10 bp, Artificial Sequence
  Synthesied
  misc_feature (1)..(10): P7-index
attggagcga

SEQ ID NO: 486 - DNA, 10 bp, Artificial Sequence
  Synthesied
  misc_feature (1)..(10): P7-index
ggacagatat

SEQ ID NO: 487 - DNA, 10 bp, Artificial Sequence
  Synthesied
  misc_feature (1)..(10): P7-index
ggacagatat

SEQ ID NO: 488 - DNA, 10 bp, Artificial Sequence
  Synthesied
  misc_feature (1)..(10): P7-index
tccttctgcc

SEQ ID NO: 489 - DNA, 10 bp, Artificial Sequence
  Synthesied
  misc_feature (1)..(10): P7-index
gccacacctt

SEQ ID NO: 490 - DNA, 10 bp, Artificial Sequence
  Synthesied
  misc_feature (1)..(10): P7-index
caagaggtag

SEQ ID NO: 491 - DNA, 10 bp, Artificial Sequence
  Synthesied
  misc_feature (1)..(10): P7-index
attcttagcc

SEQ ID NO: 492 - DNA, 10 bp, Artificial Sequence
  Synthesied
  misc_feature (1)..(10): P7-index
tggtgctaga

SEQ ID NO: 493 - DNA, 10 bp, Artificial Sequence
  Synthesied
  misc_feature (1)..(10): P7-index
acgaagttga

SEQ ID NO: 494 - DNA, 10 bp, Artificial Sequence
  Synthesied
  misc_feature (1)..(10): P7-index
tgtctagctt

SEQ ID NO: 495 - DNA, 10 bp, Artificial Sequence
  Synthesied
  misc_feature (1)..(10): P7-index
caaggtcacg

SEQ ID NO: 496 - DNA, 10 bp, Artificial Sequence
  Synthesied
  misc_feature (1)..(10): P7-index
gtctccagac

SEQ ID NO: 497 - DNA, 10 bp, Artificial Sequence
  Synthesied
  misc_feature (1)..(10): P7-index
cgagaatgtt

SEQ ID NO: 498 - DNA, 10 bp, Artificial Sequence
  Synthesied
  misc_feature (1)..(10): P7-index
aacttccaga

SEQ ID NO: 499 - DNA, 10 bp, Artificial Sequence
  Synthesied
  misc_feature (1)..(10): P7-index
tcgcgtacag

SEQ ID NO: 500 - DNA, 10 bp, Artificial Sequence
  Synthesied
  misc_feature (1)..(10): P7-index
gttacggtcc

SEQ ID NO: 501 - DNA, 10 bp, Artificial Sequence
  Synthesied
  misc_feature (1)..(10): P7-index
ggcttactag

SEQ ID NO: 502 - DNA, 10 bp, Artificial Sequence
  Synthesied
  misc_feature (1)..(10): P7-index
acagatgatc

SEQ ID NO: 503 - DNA, 10 bp, Artificial Sequence
  Synthesied
  misc_feature (1)..(10): P7-index
catcggtcca

SEQ ID NO: 504 - DNA, 10 bp, Artificial Sequence
  Synthesied
  misc_feature (1)..(10): P7-index
ttgaccaggt

SEQ ID NO: 505 - DNA, 10 bp, Artificial Sequence
  Synthesied
  misc_feature (1)..(10): P7-index
ggtatgcagg

SEQ ID NO: 506 - DNA, 10 bp, Artificial Sequence
  Synthesied
  misc_feature (1)..(10): P7-index
ctctacatac

SEQ ID NO: 507 - DNA, 10 bp, Artificial Sequence
  Synthesied
  misc_feature (1)..(10): P7-index
acacgagctt

SEQ ID NO: 508 - DNA, 10 bp, Artificial Sequence
  Synthesied
  misc_feature (1)..(10): P7-index
taggcttgca

SEQ ID NO: 509 - DNA, 10 bp, Artificial Sequence
  Synthesied
  misc_feature (1)..(10): P7-index
gagacatccg

SEQ ID NO: 510 - DNA, 10 bp, Artificial Sequence
  Synthesied
  misc_feature (1)..(10): P7-index
cctgatggac

SEQ ID NO: 511 - DNA, 10 bp, Artificial Sequence
  Synthesied
  misc_feature (1)..(10): P7-index
atctggaagt

SEQ ID NO: 512 - DNA, 10 bp, Artificial Sequence
  Synthesied
  misc_feature (1)..(10): P7-index
tgactcctta

SEQ ID NO: 513 - DNA, 10 bp, Artificial Sequence
  Synthesied
  misc_feature (1)..(10): P7-index
ctacttctgt

SEQ ID NO: 514 - DNA, 10 bp, Artificial Sequence
  Synthesied
  misc_feature (1)..(10): P7-index
agtacgtacc

SEQ ID NO: 515 - DNA, 10 bp, Artificial Sequence
  Synthesied
  misc_feature (1)..(10): P7-index
tcctgaggtg

SEQ ID NO: 516 - DNA, 10 bp, Artificial Sequence
  Synthesied
  misc_feature (1)..(10): P7-index
gaggacacaa

SEQ ID NO: 517 - DNA, 10 bp, Artificial Sequence
  Synthesied
  misc_feature (1)..(10): P7-index
tcctccatcc

SEQ ID NO: 518 - DNA, 10 bp, Artificial Sequence
  Synthesied
  misc_feature (1)..(10): P7-index
gaagaatagg

SEQ ID NO: 519 - DNA, 10 bp, Artificial Sequence
  Synthesied
  misc_feature (1)..(10): P7-index
cgtattggaa

SEQ ID NO: 520 - DNA, 10 bp, Artificial Sequence
  Synthesied
  misc_feature (1)..(10): P7-index
atgcggcctt

SEQ ID NO: 521 - DNA, 10 bp, Artificial Sequence
  Synthesied
  misc_feature (1)..(10): P7-index
aacaccttcc

SEQ ID NO: 522 - DNA, 10 bp, Artificial Sequence
  Synthesied
  misc_feature (1)..(10): P7-index
ttataagcgg

SEQ ID NO: 523 - DNA, 10 bp, Artificial Sequence
  Synthesied
  misc_feature (1)..(10): P7-index
cgtcggcaat

SEQ ID NO: 524 - DNA, 10 bp, Artificial Sequence
  Synthesied
  misc_feature (1)..(10): P7-index
gcggttagta

SEQ ID NO: 525 - DNA, 10 bp, Artificial Sequence
  Synthesied
  misc_feature (1)..(10): P7-index
gacatgcagt

SEQ ID NO: 526 - DNA, 10 bp, Artificial Sequence
  Synthesied
  misc_feature (1)..(10): P7-index
cggcgaataa

SEQ ID NO: 527 - DNA, 10 bp, Artificial Sequence
  Synthesied
  misc_feature (1)..(10): P7-index
atatatggcg

SEQ ID NO: 528 - DNA, 10 bp, Artificial Sequence
  Synthesied
  misc_feature (1)..(10): P7-index
tctgcctctc

SEQ ID NO: 529 - DNA, 10 bp, Artificial Sequence
  Synthesied
  misc_feature (1)..(10): P7-index
agtgaccgga

SEQ ID NO: 530 - DNA, 10 bp, Artificial Sequence
  Synthesied
  misc_feature (1)..(10): P7-index
gcgataatag

SEQ ID NO: 531 - DNA, 10 bp, Artificial Sequence
  Synthesied
  misc_feature (1)..(10): P7-index
ttctgttacc

SEQ ID NO: 532 - DNA, 10 bp, Artificial Sequence
  Synthesied
  misc_feature (1)..(10): P7-index
caaccggctt

SEQ ID NO: 533 - DNA, 10 bp, Artificial Sequence
  Synthesied
  misc_feature (1)..(10): P7-index
gtccattcgg

SEQ ID NO: 534 - DNA, 10 bp, Artificial Sequence
  Synthesied
  misc_feature (1)..(10): P7-index
cgaataatcc

SEQ ID NO: 535 - DNA, 10 bp, Artificial Sequence
  Synthesied
  misc_feature (1)..(10): P7-index
aattggcgaa

SEQ ID NO: 536 - DNA, 10 bp, Artificial Sequence
  Synthesied
  misc_feature (1)..(10): P7-index
tcggccgatt

SEQ ID NO: 537 - DNA, 10 bp, Artificial Sequence
  Synthesied
  misc_feature (1)..(10): P7-index
agagccgcat

SEQ ID NO: 538 - DNA, 10 bp, Artificial Sequence
  Synthesied
  misc_feature (1)..(10): P7-index
ctctgaattg

SEQ ID NO: 539 - DNA, 10 bp, Artificial Sequence
  Synthesied
  misc_feature (1)..(10): P7-index
gctaattacc

SEQ ID NO: 540 - DNA, 10 bp, Artificial Sequence
  Synthesied
  misc_feature (1)..(10): P7-index
tagctgcgga

SEQ ID NO: 541 - DNA, 10 bp, Artificial Sequence
  Synthesied
  misc_feature (1)..(10): P7-index
gatggactcc

SEQ ID NO: 542 - DNA, 10 bp, Artificial Sequence
  Synthesied
  misc_feature (1)..(10): P7-index
ttccataagg

SEQ ID NO: 543 - DNA, 10 bp, Artificial Sequence
  Synthesied
  misc_feature (1)..(10): P7-index
cgaatgtgaa

SEQ ID NO: 544 - DNA, 10 bp, Artificial Sequence
  Synthesied
  misc_feature (1)..(10): P7-index
acgtccgctt

SEQ ID NO: 545 - DNA, 10 bp, Artificial Sequence
  Synthesied
  misc_feature (1)..(10): P7-index
tatgccgcca

SEQ ID NO: 546 - DNA, 10 bp, Artificial Sequence
  Synthesied
  misc_feature (1)..(10): P7-index
atgtaacagg

SEQ ID NO: 547 - DNA, 10 bp, Artificial Sequence
  Synthesied
  misc_feature (1)..(10): P7-index
cgccttatat

SEQ ID NO: 548 - DNA, 10 bp, Artificial Sequence
  Synthesied
  misc_feature (1)..(10): P7-index
gcaaggtgtc

SEQ ID NO: 549 - DNA, 10 bp, Artificial Sequence
  Synthesied
  misc_feature (1)..(10): P7-index
acaagcgcga

SEQ ID NO: 550 - DNA, 10 bp, Artificial Sequence
  Synthesied
  misc_feature (1)..(10): P7-index
ggtccaatat

SEQ ID NO: 551 - DNA, 10 bp, Artificial Sequence
  Synthesied
  misc_feature (1)..(10): P7-index
ctggattatg

SEQ ID NO: 552 - DNA, 10 bp, Artificial Sequence
  Synthesied
  misc_feature (1)..(10): P7-index
tacttgcgcc

SEQ ID NO: 553 - DNA, 10 bp, Artificial Sequence
  Synthesied
  misc_feature (1)..(10): P7-index
gagttggcca

SEQ ID NO: 554 - DNA, 10 bp, Artificial Sequence
  Synthesied
  misc_feature (1)..(10): P7-index
cttgcacaat

SEQ ID NO: 555 - DNA, 10 bp, Artificial Sequence
  Synthesied
  misc_feature (1)..(10): P7-index
accaatatgg

SEQ ID NO: 556 - DNA, 10 bp, Artificial Sequence
  Synthesied
  misc_feature (1)..(10): P7-index
tgacgctgtc

SEQ ID NO: 557 - DNA, 10 bp, Artificial Sequence
  Synthesied
  misc_feature (1)..(10): P7-index
gaggtgtgac

SEQ ID NO: 558 - DNA, 10 bp, Artificial Sequence
  Synthesied
  misc_feature (1)..(10): P7-index
tcttcaacgt

SEQ ID NO: 559 - DNA, 10 bp, Artificial Sequence
  Synthesied
  misc_feature (1)..(10): P7-index
ataagtgtcg

SEQ ID NO: 560 - DNA, 10 bp, Artificial Sequence
  Synthesied
  misc_feature (1)..(10): P7-index
cgccaccata

SEQ ID NO: 561 - DNA, 10 bp, Artificial Sequence
  Synthesied
ggtacttact

SEQ ID NO: 562 - DNA, 10 bp, Artificial Sequence
  Synthesied
  misc_feature (1)..(10): P7-index
tagtaaggag

SEQ ID NO: 563 - DNA, 10 bp, Artificial Sequence
  Synthesied
  misc_feature (1)..(10): P7-index
acaggcactc

SEQ ID NO: 564 - DNA, 10 bp, Artificial Sequence
  Synthesied
  misc_feature (1)..(10): P7-index
ctcctgctga

SEQ ID NO: 565 - DNA, 10 bp, Artificial Sequence
  Synthesied
  misc_feature (1)..(10): P7-index
cttctagtgg

SEQ ID NO: 566 - DNA, 10 bp, Artificial Sequence
  Synthesied
  misc_feature (1)..(10): P7-index
aagaatcacc

SEQ ID NO: 567 - DNA, 10 bp, Artificial Sequence
  Synthesied
  misc_feature (1)..(10): P7-index
tcctggagaa

SEQ ID NO: 568 - DNA, 10 bp, Artificial Sequence
  Synthesied
  misc_feature (1)..(10): P7-index
ggagcctctt

SEQ ID NO: 569 - DNA, 10 bp, Artificial Sequence
  Synthesied
  misc_feature (1)..(10): P7-index
tgcataggat

SEQ ID NO: 570 - DNA, 10 bp, Artificial Sequence
  Synthesied
  misc_feature (1)..(10): P7-index
acgtataagg

SEQ ID NO: 571 - DNA, 10 bp, Artificial Sequence
  Synthesied
  misc_feature (1)..(10): P7-index
caaggcttcc

SEQ ID NO: 572 - DNA, 10 bp, Artificial Sequence
  Synthesied
  misc_feature (1)..(10): P7-index
gttccgccta

SEQ ID NO: 573 - DNA, 10 bp, Artificial Sequence
  Synthesied
  misc_feature (1)..(10): P7-index
tgtccgagag

SEQ ID NO: 574 - DNA, 10 bp, Artificial Sequence
  Synthesied
  misc_feature (1)..(10): P7-index
aaggacgtgc

SEQ ID NO: 575 - DNA, 10 bp, Artificial Sequence
  Synthesied
  misc_feature (1)..(10): P7-index
ctcatatcca

SEQ ID NO: 576 - DNA, 10 bp, Artificial Sequence
  Synthesied
  misc_feature (1)..(10): P7-index
gcatgtcatt

SEQ ID NO: 577 - DNA, 10 bp, Artificial Sequence
  Synthesied
  misc_feature (1)..(10): P7-index
tctatcgcat

SEQ ID NO: 578 - DNA, 10 bp, Artificial Sequence
  Synthesied
  misc_feature (1)..(10): P7-index
gaccgaatta

SEQ ID NO: 579 - DNA, 10 bp, Artificial Sequence
  Synthesied
  misc_feature (1)..(10): P7-index
cgagcttagg

SEQ ID NO: 580 - DNA, 10 bp, Artificial Sequence
  Synthesied
  misc_feature (1)..(10): P7-index
atgtagcgcc

SEQ ID NO: 581 - DNA, 10 bp, Artificial Sequence
  Synthesied
  misc_feature (1)..(10): P7-index
ttcgctgacc

SEQ ID NO: 582 - DNA, 10 bp, Artificial Sequence
  Synthesied
  misc_feature (1)..(10): P7-index
gagtagctaa

SEQ ID NO: 583 - DNA, 10 bp, Artificial Sequence
  Synthesied
  misc_feature (1)..(10): P7-index
acactaagtg

SEQ ID NO: 584 - DNA, 10 bp, Artificial Sequence
  Synthesied
  misc_feature (1)..(10): P7-index
cgtagctcgt

SEQ ID NO: 585 - DNA, 10 bp, Artificial Sequence
  Synthesied
  misc_feature (1)..(10): P7-index
aactacagcc

SEQ ID NO: 586 - DNA, 10 bp, Artificial Sequence
  Synthesied
  misc_feature (1)..(10): P7-index
ccgctattgg

SEQ ID NO: 587 - DNA, 10 bp, Artificial Sequence
  Synthesied
  misc_feature (1)..(10): P7-index
ttaaggccaa

SEQ ID NO: 588 - DNA, 10 bp, Artificial Sequence
  Synthesied
  misc_feature (1)..(10): P7-index
ggtgctgatt

SEQ ID NO: 589 - DNA, 10 bp, Artificial Sequence
  Synthesied
  misc_feature (1)..(10): P7-index
cggttcgttc

SEQ ID NO: 590 - DNA, 10 bp, Artificial Sequence
  Synthesied
  misc_feature (1)..(10): P7-index
actcgaccga

SEQ ID NO: 591 - DNA, 10 bp, Artificial Sequence
  Synthesied
  misc_feature (1)..(10): P7-index
taagagaacg

SEQ ID NO: 592 - DNA, 10 bp, Artificial Sequence
  Synthesied
  misc_feature (1)..(10): P7-index
gtcacttgat

SEQ ID NO: 593 - DNA, 10 bp, Artificial Sequence
  Synthesied
  misc_feature (1)..(10): P7-index
aagaccgtcg

SEQ ID NO: 594 - DNA, 10 bp, Artificial Sequence
  Synthesied
  misc_feature (1)..(10): P7-index
gcctaacgga

SEQ ID NO: 595 - DNA, 10 bp, Artificial Sequence
  Synthesied
  misc_feature (1)..(10): P7-index
ttagtgacac

SEQ ID NO: 596 - DNA, 10 bp, Artificial Sequence
  Synthesied
  misc_feature (1)..(10): P7-index
cgtcgttatt

SEQ ID NO: 597 - DNA, 10 bp, Artificial Sequence
  Synthesied
  misc_feature (1)..(10): P7-index
tgacgccaga

SEQ ID NO: 598 - DNA, 10 bp, Artificial Sequence
  Synthesied
  misc_feature (1)..(10): P7-index
cctaatagct

SEQ ID NO: 599 - DNA, 10 bp, Artificial Sequence
  Synthesied
  misc_feature (1)..(10): P7-index
gagttatcag

SEQ ID NO: 600 - DNA, 10 bp, Artificial Sequence
  Synthesied
  misc_feature (1)..(10): P7-index
atcgcggttc

SEQ ID NO: 601 - DNA, 10 bp, Artificial Sequence
  Synthesied
  misc_feature (1)..(10): P7-index
aacctgcgct

SEQ ID NO: 602 - DNA, 10 bp, Artificial Sequence
  Synthesied
  misc_feature (1)..(10): P7-index
cggtcatatg

SEQ ID NO: 603 - DNA, 10 bp, Artificial Sequence
  Synthesied
  misc_feature (1)..(10): P7-index
ttaagtacgc

SEQ ID NO: 604 - DNA, 10 bp, Artificial Sequence
  Synthesied
  misc_feature (1)..(10): P7-index
gctgacgtaa

SEQ ID NO: 605 - DNA, 10 bp, Artificial Sequence
  Synthesied
  misc_feature (1)..(10): P7-index
cactgcatgg

SEQ ID NO: 606 - DNA, 10 bp, Artificial Sequence
  Synthesied
  misc_feature (1)..(10): P7-index
ataacagacc

SEQ ID NO: 607 - DNA, 10 bp, Artificial Sequence
  Synthesied
  misc_feature (1)..(10): P7-index
tgtgatcgaa

SEQ ID NO: 608 - DNA, 10 bp, Artificial Sequence
  Synthesied
  misc_feature (1)..(10): P7-index
gcgctgtctt

SEQ ID NO: 609 - DNA, 10 bp, Artificial Sequence
  Synthesied
  misc_feature (1)..(10): P7-index
tgttctaccg

SEQ ID NO: 610 - DNA, 10 bp, Artificial Sequence
  Synthesied
  misc_feature (1)..(10): P7-index
ccggaatatc

SEQ ID NO: 611 - DNA, 10 bp, Artificial Sequence
  Synthesied
  misc_feature (1)..(10): P7-index
gacatggtaa

SEQ ID NO: 612 - DNA, 10 bp, Artificial Sequence
  Synthesied
  misc_feature (1)..(10): P7-index
atacgccggt

SEQ ID NO: 613 - DNA, 10 bp, Artificial Sequence
  Synthesied
  misc_feature (1)..(10): P7-index
aggattcgcc

SEQ ID NO: 614 - DNA, 10 bp, Artificial Sequence
  Synthesied
  misc_feature (1)..(10): P7-index
taatgagtgg

SEQ ID NO: 615 - DNA, 10 bp, Artificial Sequence
  Synthesied
  misc_feature (1)..(10): P7-index
gctgcgaatt

SEQ ID NO: 616 - DNA, 10 bp, Artificial Sequence
  Synthesied
  misc_feature (1)..(10): P7-index
ctccactcaa

SEQ ID NO: 617 - DNA, 10 bp, Artificial Sequence
  Synthesied
  misc_feature (1)..(10): P7-index
tgcctaccag

SEQ ID NO: 618 - DNA, 10 bp, Artificial Sequence
  Synthesied
  misc_feature (1)..(10): P7-index
ccgagtaatt

SEQ ID NO: 619 - DNA, 10 bp, Artificial Sequence
  Synthesied
  misc_feature (1)..(10): P7-index
attgagttgc

SEQ ID NO: 620 - DNA, 10 bp, Artificial Sequence
  Synthesied
  misc_feature (1)..(10): P7-index
gaatccggca

SEQ ID NO: 621 - DNA, 10 bp, Artificial Sequence
  Synthesied
  misc_feature (1)..(10): P7-index
gactgactgc

SEQ ID NO: 622 - DNA, 10 bp, Artificial Sequence
  Synthesied
  misc_feature (1)..(10): P7-index
agtgctacat

SEQ ID NO: 623 - DNA, 10 bp, Artificial Sequence
  Synthesied
  misc_feature (1)..(10): P7-index
ccaatgtatg

SEQ ID NO: 624 - DNA, 10 bp, Artificial Sequence
  Synthesied
  misc_feature (1)..(10): P7-index
ttgcacggca

SEQ ID NO: 625 - DNA, 10 bp, Artificial Sequence
  Synthesied
  misc_feature (1)..(10): P7-index
aggccagtct

SEQ ID NO: 626 - DNA, 10 bp, Artificial Sequence
  Synthesied
  misc_feature (1)..(10): P7-index
ccaattcaag

SEQ ID NO: 627 - DNA, 10 bp, Artificial Sequence
  Synthesied
  misc_feature (1)..(10): P7-index
gattagagtc

SEQ ID NO: 628 - DNA, 10 bp, Artificial Sequence
  Synthesied
  misc_feature (1)..(10): P7-index
ttcggctcga

SEQ ID NO: 629 - DNA, 10 bp, Artificial Sequence
  Synthesied
  misc_feature (1)..(10): P7-index
aggcttaagt

SEQ ID NO: 630 - DNA, 10 bp, Artificial Sequence
  Synthesied
  misc_feature (1)..(10): P7-index
taatgctccg

SEQ ID NO: 631 - DNA, 10 bp, Artificial Sequence
  Synthesied
  misc_feature (1)..(10): P7-index
gtcgaggtaa

SEQ ID NO: 632 - DNA, 10 bp, Artificial Sequence
  Synthesied
  misc_feature (1)..(10): P7-index
cctacacgtc

SEQ ID NO: 633 - DNA, 10 bp, Artificial Sequence
  Synthesied
  misc_feature (1)..(10): P7-index
tgaccaccga

SEQ ID NO: 634 - DNA, 10 bp, Artificial Sequence
  Synthesied
  misc_feature (1)..(10): P7-index
gataaggatc

SEQ ID NO: 635 - DNA, 10 bp, Artificial Sequence
  Synthesied
  misc_feature (1)..(10): P7-index
ctgttcatag

SEQ ID NO: 636 - DNA, 10 bp, Artificial Sequence
  Synthesied
  misc_feature (1)..(10): P7-index
accggttgct

SEQ ID NO: 637 - DNA, 10 bp, Artificial Sequence
  Synthesied
  misc_feature (1)..(10): P7-index
ctcaggacta

SEQ ID NO: 638 - DNA, 10 bp, Artificial Sequence
  Synthesied
  misc_feature (1)..(10): P7-index
aattcacgcc

SEQ ID NO: 639 - DNA, 10 bp, Artificial Sequence
  Synthesied
  misc_feature (1)..(10): P7-index
ggagattaag

SEQ ID NO: 640 - DNA, 10 bp, Artificial Sequence
  Synthesied
  misc_feature (1)..(10): P7-index
tcgctcgtgt

SEQ ID NO: 641 - DNA, 10 bp, Artificial Sequence
  Synthesied
  misc_feature (1)..(10): P7-index
aaggtccgca

SEQ ID NO: 642 - DNA, 10 bp, Artificial Sequence
  Synthesied
  misc_feature (1)..(10): P7-index
gtcaatacgt

SEQ ID NO: 643 - DNA, 10 bp, Artificial Sequence
  Synthesied
  misc_feature (1)..(10): P7-index
cgatgatatc

SEQ ID NO: 644 - DNA, 10 bp, Artificial Sequence
  Synthesied
  misc_feature (1)..(10): P7-index
tctccggtag

SEQ ID NO: 645 - DNA, 10 bp, Artificial Sequence
  Synthesied
  misc_feature (1)..(10): P7-index
atgcgtgcac

SEQ ID NO: 646 - DNA, 10 bp, Artificial Sequence
  Synthesied
  misc_feature (1)..(10): P7-index
tatgcgtgtg

SEQ ID NO: 647 - DNA, 10 bp, Artificial Sequence
  Synthesied
  misc_feature (1)..(10): P7-index
gccaacaaga

SEQ ID NO: 648 - DNA, 10 bp, Artificial Sequence
  Synthesied
  misc_feature (1)..(10): P7-index
cgattactct

SEQ ID NO: 649 - DNA, 10 bp, Artificial Sequence
  Synthesied
  misc_feature (1)..(10): P7-index
ttcggccaca

SEQ ID NO: 650 - DNA, 10 bp, Artificial Sequence
  Synthesied
  misc_feature (1)..(10): P7-index
gaatctggtg

SEQ ID NO: 651 - DNA, 10 bp, Artificial Sequence
  Synthesied
  misc_feature (1)..(10): P7-index
cgtaagatac

SEQ ID NO: 652 - DNA, 10 bp, Artificial Sequence
  Synthesied
  misc_feature (1)..(10): P7-index
acgctatcgt

SEQ ID NO: 653 - DNA, 10 bp, Artificial Sequence
  Synthesied
  misc_feature (1)..(10): P7-index
gattcgcgag

SEQ ID NO: 654 - DNA, 10 bp, Artificial Sequence
  Synthesied
  misc_feature (1)..(10): P7-index
ctcaacgtcc

SEQ ID NO: 655 - DNA, 10 bp, Artificial Sequence
  Synthesied
  misc_feature (1)..(10): P7-index
tcggtaacta

SEQ ID NO: 656 - DNA, 10 bp, Artificial Sequence
  Synthesied
  misc_feature (1)..(10): P7-index
agacgttagt

SEQ ID NO: 657 - DNA, 10 bp, Artificial Sequence
  Synthesied
  misc_feature (1)..(10): P7-index
gatccgttcc

SEQ ID NO: 658 - DNA, 10 bp, Artificial Sequence
  Synthesied
  misc_feature (1)..(10): P7-index
ctcttcagaa

SEQ ID NO: 659 - DNA, 10 bp, Artificial Sequence
  Synthesied
  misc_feature (1)..(10): P7-index
agaagagatg

SEQ ID NO: 660 - DNA, 10 bp, Artificial Sequence
  Synthesied
  misc_feature (1)..(10): P7-index
tcggatccgt

SEQ ID NO: 661 - DNA, 10 bp, Artificial Sequence
  Synthesied
  misc_feature (1)..(10): P7-index
ttgccttgcg

SEQ ID NO: 662 - DNA, 10 bp, Artificial Sequence
  Synthesied
  misc_feature (1)..(10): P7-index
gaagtaccga

SEQ ID NO: 663 - DNA, 10 bp, Artificial Sequence
  Synthesied
  misc_feature (1)..(10): P7-index
ccttggaatc

SEQ ID NO: 664 - DNA, 10 bp, Artificial Sequence
  Synthesied
  misc_feature (1)..(10): P7-index
agcaacgtat

SEQ ID NO: 665 - DNA, 10 bp, Artificial Sequence
  Synthesied
  misc_feature (1)..(10): P7-index
gactgtcgag

SEQ ID NO: 666 - DNA, 10 bp, Artificial Sequence
  Synthesied
  misc_feature (1)..(10): P7-index
ctaacagtgc

SEQ ID NO: 667 - DNA, 10 bp, Artificial Sequence
  Synthesied
  misc_feature (1)..(10): P7-index
tcggagaaca

SEQ ID NO: 668 - DNA, 10 bp, Artificial Sequence
  Synthesied
  misc_feature (1)..(10): P7-index
agtctctctt

SEQ ID NO: 669 - DNA, 10 bp, Artificial Sequence
  Synthesied
  misc_feature (1)..(10): P7-index
atggacggac

SEQ ID NO: 670 - DNA, 10 bp, Artificial Sequence
  Synthesied
  misc_feature (1)..(10): P7-index
ccatcatcta

SEQ ID NO: 671 - DNA, 10 bp, Artificial Sequence
  Synthesied
  misc_feature (1)..(10): P7-index
tatcttcacg

SEQ ID NO: 672 - DNA, 10 bp, Artificial Sequence
  Synthesied
ggcaggatgt

SEQ ID NO: 673 - DNA, 10 bp, Artificial Sequence
  Synthesied
  misc_feature (1)..(10): P7-index
atgtgcacta

SEQ ID NO: 674 - DNA, 10 bp, Artificial Sequence
  Synthesied
  misc_feature (1)..(10): P7-index
taagcgcacc

SEQ ID NO: 675 - DNA, 10 bp, Artificial Sequence
  Synthesied
  misc_feature (1)..(10): P7-index
cctcaatgat

SEQ ID NO: 676 - DNA, 10 bp, Artificial Sequence
  Synthesied
  misc_feature (1)..(10): P7-index
ggcattgtgg

SEQ ID NO: 677 - DNA, 10 bp, Artificial Sequence
  Synthesied
  misc_feature (1)..(10): P7-index
gcagccacaa

SEQ ID NO: 678 - DNA, 10 bp, Artificial Sequence
  Synthesied
  misc_feature (1)..(10): P7-index
caccaattct

SEQ ID NO: 679 - DNA, 10 bp, Artificial Sequence
  Synthesied
  misc_feature (1)..(10): P7-index
atgatggatg

SEQ ID NO: 680 - DNA, 10 bp, Artificial Sequence
  Synthesied
  misc_feature (1)..(10): P7-index
tgttgtcggc

SEQ ID NO: 681 - DNA, 10 bp, Artificial Sequence
  Synthesied
  misc_feature (1)..(10): P7-index
ctctgagcta

SEQ ID NO: 682 - DNA, 10 bp, Artificial Sequence
  Synthesied
  misc_feature (1)..(10): P7-index
ggaatcctgt

SEQ ID NO: 683 - DNA, 10 bp, Artificial Sequence
  Synthesied
  misc_feature (1)..(10): P7-index
aatccgaacg

SEQ ID NO: 684 - DNA, 10 bp, Artificial Sequence
  Synthesied
  misc_feature (1)..(10): P7-index
tcggattgac

SEQ ID NO: 685 - DNA, 10 bp, Artificial Sequence
  Synthesied
  misc_feature (1)..(10): P7-index
taccgataac

SEQ ID NO: 686 - DNA, 10 bp, Artificial Sequence
  Synthesied
  misc_feature (1)..(10): P7-index
gcgtctatta

SEQ ID NO: 687 - DNA, 10 bp, Artificial Sequence
  Synthesied
  misc_feature (1)..(10): P7-index
ctagaggcgt

SEQ ID NO: 688 - DNA, 10 bp, Artificial Sequence
  Synthesied
  misc_feature (1)..(10): P7-index
agtatccgcg

SEQ ID NO: 689 - DNA, 10 bp, Artificial Sequence
  Synthesied
  misc_feature (1)..(10): P7-index
cattgccata

SEQ ID NO: 690 - DNA, 10 bp, Artificial Sequence
  Synthesied
  misc_feature (1)..(10): P7-index
ggacttggct

SEQ ID NO: 691 - DNA, 10 bp, Artificial Sequence
  Synthesied
  misc_feature (1)..(10): P7-index
ttgacgatac

SEQ ID NO: 692 - DNA, 10 bp, Artificial Sequence
  Synthesied
  misc_feature (1)..(10): P7-index
accgaatcgg

SEQ ID NO: 693 - DNA, 10 bp, Artificial Sequence
  Synthesied
  misc_feature (1)..(10): P7-index
tcagaactcc

SEQ ID NO: 694 - DNA, 10 bp, Artificial Sequence
  Synthesied
  misc_feature (1)..(10): P7-index
ggcacgaata

SEQ ID NO: 695 - DNA, 10 bp, Artificial Sequence
  Synthesied
  misc_feature (1)..(10): P7-index
cttcttgcag

SEQ ID NO: 696 - DNA, 10 bp, Artificial Sequence
  Synthesied
  misc_feature (1)..(10): P7-index
aagtgctggt

SEQ ID NO: 697 - DNA, 10 bp, Artificial Sequence
  Synthesied
  misc_feature (1)..(10): P7-index
taggcactag

SEQ ID NO: 698 - DNA, 10 bp, Artificial Sequence
  Synthesied
  misc_feature (1)..(10): P7-index
ggtctctgta

SEQ ID NO: 699 - DNA, 10 bp, Artificial Sequence
  Synthesied
  misc_feature (1)..(10): P7-index
ctatgtaagc

SEQ ID NO: 700 - DNA, 10 bp, Artificial Sequence
  Synthesied
  misc_feature (1)..(10): P7-index
accaaggcct

SEQ ID NO: 701 - DNA, 10 bp, Artificial Sequence
  Synthesied
  misc_feature (1)..(10): P7-index
tgaactcgcg

SEQ ID NO: 702 - DNA, 10 bp, Artificial Sequence
  Synthesied
  misc_feature (1)..(10): P7-index
acttaggcgc

SEQ ID NO: 703 - DNA, 10 bp, Artificial Sequence
  Synthesied
  misc_feature (1)..(10): P7-index
gaggtcaatt

SEQ ID NO: 704 - DNA, 10 bp, Artificial Sequence
  Synthesied
  misc_feature (1)..(10): P7-index
ctccgattaa

SEQ ID NO: 705 - DNA, 10 bp, Artificial Sequence
  Synthesied
  misc_feature (1)..(10): P7-index
cacgatacta

SEQ ID NO: 706 - DNA, 10 bp, Artificial Sequence
  Synthesied
  misc_feature (1)..(10): P7-index
acactatacc

SEQ ID NO: 707 - DNA, 10 bp, Artificial Sequence
  Synthesied
  misc_feature (1)..(10): P7-index
ttgaggcgag

SEQ ID NO: 708 - DNA, 10 bp, Artificial Sequence
  Synthesied
  misc_feature (1)..(10): P7-index
ggttccgtgt

SEQ ID NO: 709 - DNA, 10 bp, Artificial Sequence
  Synthesied
  misc_feature (1)..(10): P7-index
tgcacgaacc

SEQ ID NO: 710 - DNA, 10 bp, Artificial Sequence
  Synthesied
  misc_feature (1)..(10): P7-index
gattgtgctg

SEQ ID NO: 711 - DNA, 10 bp, Artificial Sequence
  Synthesied
  misc_feature (1)..(10): P7-index
atgctcttga

SEQ ID NO: 712 - DNA, 10 bp, Artificial Sequence
  Synthesied
  misc_feature (1)..(10): P7-index
ccagaacgat

SEQ ID NO: 713 - DNA, 10 bp, Artificial Sequence
  Synthesied
  misc_feature (1)..(10): P7-index
gagctagaac

SEQ ID NO: 714 - DNA, 10 bp, Artificial Sequence
  Synthesied
  misc_feature (1)..(10): P7-index
actagttggt

SEQ ID NO: 715 - DNA, 10 bp, Artificial Sequence
  Synthesied
  misc_feature (1)..(10): P7-index
ttagcgcttg

SEQ ID NO: 716 - DNA, 10 bp, Artificial Sequence
  Synthesied
  misc_feature (1)..(10): P7-index
cgctacacca

SEQ ID NO: 717 - DNA, 10 bp, Artificial Sequence
  Synthesied
  misc_feature (1)..(10): P7-index
tgtcgacacc

SEQ ID NO: 718 - DNA, 10 bp, Artificial Sequence
  Synthesied
  misc_feature (1)..(10): P7-index
gcaatcttag

SEQ ID NO: 719 - DNA, 10 bp, Artificial Sequence
  Synthesied
  misc_feature (1)..(10): P7-index
cagtatggta

SEQ ID NO: 720 - DNA, 10 bp, Artificial Sequence
  Synthesied
  misc_feature (1)..(10): P7-index
atcgcgacgt

SEQ ID NO: 721 - DNA, 10 bp, Artificial Sequence
  Synthesied
  misc_feature (1)..(10): P7-index
cgttgcggat

SEQ ID NO: 722 - DNA, 10 bp, Artificial Sequence
  Synthesied
  misc_feature (1)..(10): P7-index
aagcagcagg

SEQ ID NO: 723 - DNA, 10 bp, Artificial Sequence
  Synthesied
  misc_feature (1)..(10): P7-index
ttcactactc

SEQ ID NO: 724 - DNA, 10 bp, Artificial Sequence
  Synthesied
  misc_feature (1)..(10): P7-index
gcagtattca

SEQ ID NO: 725 - DNA, 10 bp, Artificial Sequence
  Synthesied
  misc_feature (1)..(10): P7-index
atgcatcaac

SEQ ID NO: 726 - DNA, 10 bp, Artificial Sequence
  Synthesied
  misc_feature (1)..(10): P7-index
tacgtagtct

SEQ ID NO: 727 - DNA, 10 bp, Artificial Sequence
  Synthesied
  misc_feature (1)..(10): P7-index
ggtaggtcga

SEQ ID NO: 728 - DNA, 10 bp, Artificial Sequence
  Synthesied
  misc_feature (1)..(10): P7-index
ccatccagtg

SEQ ID NO: 729 - DNA, 10 bp, Artificial Sequence
  Synthesied
  misc_feature (1)..(10): P7-index
gaccacgatc

SEQ ID NO: 730 - DNA, 10 bp, Artificial Sequence
  Synthesied
  misc_feature (1)..(10): P7-index
ctaatacgag

SEQ ID NO: 731 - DNA, 10 bp, Artificial Sequence
  Synthesied
  misc_feature (1)..(10): P7-index
agttgtacga

SEQ ID NO: 732 - DNA, 10 bp, Artificial Sequence
  Synthesied
  misc_feature (1)..(10): P7-index
tcggcgttct

SEQ ID NO: 733 - DNA, 10 bp, Artificial Sequence
  Synthesied
  misc_feature (1)..(10): P7-index
cggtgagcaa

SEQ ID NO: 734 - DNA, 10 bp, Artificial Sequence
  Synthesied
  misc_feature (1)..(10): P7-index
aataaccacg

SEQ ID NO: 735 - DNA, 10 bp, Artificial Sequence
  Synthesied
  misc_feature (1)..(10): P7-index
ttcgttatgc

SEQ ID NO: 736 - DNA, 10 bp, Artificial Sequence
  Synthesied
  misc_feature (1)..(10): P7-index
gcaccgtgtt

SEQ ID NO: 737 - DNA, 10 bp, Artificial Sequence
  Synthesied
  misc_feature (1)..(10): P7-index
ccaacgactg

SEQ ID NO: 738 - DNA, 10 bp, Artificial Sequence
  Synthesied
  misc_feature (1)..(10): P7-index
agcttctaac

SEQ ID NO: 739 - DNA, 10 bp, Artificial Sequence
  Synthesied
  misc_feature (1)..(10): P7-index
tatgaaggca

SEQ ID NO: 740 - DNA, 10 bp, Artificial Sequence
  Synthesied
  misc_feature (1)..(10): P7-index
gtgcgtctgt

SEQ ID NO: 741 - DNA, 10 bp, Artificial Sequence
  Synthesied
  misc_feature (1)..(10): P7-index
ggtggaacac

SEQ ID NO: 742 - DNA, 10 bp, Artificial Sequence
  Synthesied
  misc_feature (1)..(10): P7-index
ttgtatcgtg

SEQ ID NO: 743 - DNA, 10 bp, Artificial Sequence
  Synthesied
  misc_feature (1)..(10): P7-index
caactgtaga

SEQ ID NO: 744 - DNA, 10 bp, Artificial Sequence
  Synthesied
  misc_feature (1)..(10): P7-index
accaccgtct

SEQ ID NO: 745 - DNA, 10 bp, Artificial Sequence
  Synthesied
  misc_feature (1)..(10): P7-index
caggctgttc

SEQ ID NO: 746 - DNA, 10 bp, Artificial Sequence
  Synthesied
  misc_feature (1)..(10): P7-index
tgcaggaaga

SEQ ID NO: 747 - DNA, 10 bp, Artificial Sequence
  Synthesied
  misc_feature (1)..(10): P7-index
gtataacgct

SEQ ID NO: 748 - DNA, 10 bp, Artificial Sequence
  Synthesied
  misc_feature (1)..(10): P7-index
actctctcag

SEQ ID NO: 749 - DNA, 10 bp, Artificial Sequence
  Synthesied
  misc_feature (1)..(10): P7-index
cggtgaacct

SEQ ID NO: 750 - DNA, 10 bp, Artificial Sequence
  Synthesied
  misc_feature (1)..(10): P7-index
acaattggag

SEQ ID NO: 751 - DNA, 10 bp, Artificial Sequence
  Synthesied
  misc_feature (1)..(10): P7-index
gatgcgtata

SEQ ID NO: 752 - DNA, 10 bp, Artificial Sequence
  Synthesied
  misc_feature (1)..(10): P7-index
ttccacctgc

SEQ ID NO: 753 - DNA, 10 bp, Artificial Sequence
  Synthesied
  misc_feature (1)..(10): P7-index
gtccacagga

SEQ ID NO: 754 - DNA, 10 bp, Artificial Sequence
  Synthesied
  misc_feature (1)..(10): P7-index
tgaatacctc

SEQ ID NO: 755 - DNA, 10 bp, Artificial Sequence
  Synthesied
  misc_feature (1)..(10): P7-index
cattgttacg

SEQ ID NO: 756 - DNA, 10 bp, Artificial Sequence
  Synthesied
  misc_feature (1)..(10): P7-index
acggcggtat

SEQ ID NO: 757 - DNA, 10 bp, Artificial Sequence
  Synthesied
  misc_feature (1)..(10): P7-index
actgcgctag

SEQ ID NO: 758 - DNA, 10 bp, Artificial Sequence
  Synthesied
  misc_feature (1)..(10): P7-index
caattctcga

SEQ ID NO: 759 - DNA, 10 bp, Artificial Sequence
  Synthesied
  misc_feature (1)..(10): P7-index
ttgagaagcc

SEQ ID NO: 760 - DNA, 10 bp, Artificial Sequence
  Synthesied
  misc_feature (1)..(10): P7-index
ggccatgatt

SEQ ID NO: 761 - DNA, 10 bp, Artificial Sequence
  Synthesied
  misc_feature (1)..(10): P7-index
aggcactgtt

SEQ ID NO: 762 - DNA, 10 bp, Artificial Sequence
  Synthesied
  misc_feature (1)..(10): P7-index
gtcataacag

SEQ ID NO: 763 - DNA, 10 bp, Artificial Sequence
  Synthesied
  misc_feature (1)..(10): P7-index
taaggtgagc

SEQ ID NO: 764 - DNA, 10 bp, Artificial Sequence
  Synthesied
  misc_feature (1)..(10): P7-index
ccttcgctca

SEQ ID NO: 765 - DNA, 10 bp, Artificial Sequence
  Synthesied
  misc_feature (1)..(10): P7-index
ctcgtgtagg

SEQ ID NO: 766 - DNA, 10 bp, Artificial Sequence
  Synthesied
  misc_feature (1)..(10): P7-index
agaagaacct

SEQ ID NO: 767 - DNA, 10 bp, Artificial Sequence
  Synthesied
  misc_feature (1)..(10): P7-index
tattctggtc

SEQ ID NO: 768 - DNA, 10 bp, Artificial Sequence
  Synthesied
  misc_feature (1)..(10): P7-index
gcgcacctaa

SEQ ID NO: 769 - DNA, 10 bp, Artificial Sequence
  Synthesied
  misc_feature (1)..(10): P7-index
tacgtggacc

SEQ ID NO: 770 - DNA, 10 bp, Artificial Sequence
  Synthesied
  misc_feature (1)..(10): P7-index
ccaagatgaa

SEQ ID NO: 771 - DNA, 10 bp, Artificial Sequence
  Synthesied
  misc_feature (1)..(10): P7-index
gttcatcttg

SEQ ID NO: 772 - DNA, 10 bp, Artificial Sequence
  Synthesied
  misc_feature (1)..(10): P7-index
aggtccacgt

SEQ ID NO: 773 - DNA, 10 bp, Artificial Sequence
  Synthesied
  misc_feature (1)..(10): P7-index
cgtgtgtctc

SEQ ID NO: 774 - DNA, 10 bp, Artificial Sequence
  Synthesied
  misc_feature (1)..(10): P7-index
acacgtgaat

SEQ ID NO: 775 - DNA, 10 bp, Artificial Sequence
  Synthesied
  misc_feature (1)..(10): P7-index
tagaacatgg

SEQ ID NO: 776 - DNA, 10 bp, Artificial Sequence
  Synthesied
  misc_feature (1)..(10): P7-index
gtctcacgca

SEQ ID NO: 777 - DNA, 10 bp, Artificial Sequence
  Synthesied
  misc_feature (1)..(10): P7-index
ccatgcggaa

SEQ ID NO: 778 - DNA, 10 bp, Artificial Sequence
  Synthesied
  misc_feature (1)..(10): P7-index
tatacgactc

SEQ ID NO: 779 - DNA, 10 bp, Artificial Sequence
  Synthesied
  misc_feature (1)..(10): P7-index
gtggaattct

SEQ ID NO: 780 - DNA, 10 bp, Artificial Sequence
  Synthesied
  misc_feature (1)..(10): P7-index
agccttcagg

SEQ ID NO: 781 - DNA, 10 bp, Artificial Sequence
  Synthesied
  misc_feature (1)..(10): P7-index
ctgtgttcag

SEQ ID NO: 782 - DNA, 10 bp, Artificial Sequence
  Synthesied
  misc_feature (1)..(10): P7-index
aatgcgcgct

SEQ ID NO: 783 - DNA, 10 bp, Artificial Sequence
  Synthesied
  misc_feature (1)..(10): P7-index
tcacaagatc

SEQ ID NO: 784 - DNA, 10 bp, Artificial Sequence
  Synthesied
  misc_feature (1)..(10): P7-index
ggcatcatga

SEQ ID NO: 785 - DNA, 10 bp, Artificial Sequence
  Synthesied
  misc_feature (1)..(10): P7-index
tggagtacgg

SEQ ID NO: 786 - DNA, 10 bp, Artificial Sequence
  Synthesied
  misc_feature (1)..(10): P7-index
gaactgcatt

SEQ ID NO: 787 - DNA, 10 bp, Artificial Sequence
  Synthesied
  misc_feature (1)..(10): P7-index
cttgacttcc

SEQ ID NO: 788 - DNA, 10 bp, Artificial Sequence
  Synthesied
  misc_feature (1)..(10): P7-index
acctcaggaa

SEQ ID NO: 789 - DNA, 10 bp, Artificial Sequence
  Synthesied
  misc_feature (1)..(10): P7-index
ttcacgcaca

SEQ ID NO: 790 - DNA, 10 bp, Artificial Sequence
  Synthesied
  misc_feature (1)..(10): P7-index
gaacgtaggt

SEQ ID NO: 791 - DNA, 10 bp, Artificial Sequence
  Synthesied
  misc_feature (1)..(10): P7-index
cgttaagctg

SEQ ID NO: 792 - DNA, 10 bp, Artificial Sequence
  Synthesied
acggtcttac

SEQ ID NO: 793 - DNA, 10 bp, Artificial Sequence
  Synthesied
  misc_feature (1)..(10): P7-index
tcttgtgact

SEQ ID NO: 794 - DNA, 10 bp, Artificial Sequence
  Synthesied
  misc_feature (1)..(10): P7-index
gaaccgatgg

SEQ ID NO: 795 - DNA, 10 bp, Artificial Sequence
  Synthesied
  misc_feature (1)..(10): P7-index
ctgaaccgac

SEQ ID NO: 796 - DNA, 10 bp, Artificial Sequence
  Synthesied
  misc_feature (1)..(10): P7-index
agcgtatcta

SEQ ID NO: 797 - DNA, 10 bp, Artificial Sequence
  Synthesied
  misc_feature (1)..(10): P7-index
tacctcactc

SEQ ID NO: 798 - DNA, 10 bp, Artificial Sequence
  Synthesied
  misc_feature (1)..(10): P7-index
agagatcggt

SEQ ID NO: 799 - DNA, 10 bp, Artificial Sequence
  Synthesied
  misc_feature (1)..(10): P7-index
gttaggttag

SEQ ID NO: 800 - DNA, 10 bp, Artificial Sequence
  Synthesied
  misc_feature (1)..(10): P7-index
ccgtcagaca

SEQ ID NO: 801 - DNA, 10 bp, Artificial Sequence
  Synthesied
  misc_feature (1)..(10): P7-index
gtgctaagtc

SEQ ID NO: 802 - DNA, 10 bp, Artificial Sequence
  Synthesied
  misc_feature (1)..(10): P7-index
tctacgttca

SEQ ID NO: 803 - DNA, 10 bp, Artificial Sequence
  Synthesied
  misc_feature (1)..(10): P7-index
aactgtgcgt

SEQ ID NO: 804 - DNA, 10 bp, Artificial Sequence
  Synthesied
  misc_feature (1)..(10): P7-index
cgagaccaag

SEQ ID NO: 805 - DNA, 10 bp, Artificial Sequence
  Synthesied
  misc_feature (1)..(10): P7-index
cacggttctt

SEQ ID NO: 806 - DNA, 10 bp, Artificial Sequence
  Synthesied
  misc_feature (1)..(10): P7-index
atacaggagg

SEQ ID NO: 807 - DNA, 10 bp, Artificial Sequence
  Synthesied
  misc_feature (1)..(10): P7-index
gcgatacgac

SEQ ID NO: 808 - DNA, 10 bp, Artificial Sequence
  Synthesied
  misc_feature (1)..(10): P7-index
tgttccatca

SEQ ID NO: 809 - DNA, 10 bp, Artificial Sequence
  Synthesied
  misc_feature (1)..(10): P7-index
agatctcagc

SEQ ID NO: 810 - DNA, 10 bp, Artificial Sequence
  Synthesied
  misc_feature (1)..(10): P7-index
cctatgagtt

SEQ ID NO: 811 - DNA, 10 bp, Artificial Sequence
  Synthesied
  misc_feature (1)..(10): P7-index
gtcggcttaa

SEQ ID NO: 812 - DNA, 10 bp, Artificial Sequence
  Synthesied
  misc_feature (1)..(10): P7-index
tagcaagccg

SEQ ID NO: 813 - DNA, 10 bp, Artificial Sequence
  Synthesied
  misc_feature (1)..(10): P7-index
cagtctagga

SEQ ID NO: 814 - DNA, 10 bp, Artificial Sequence
  Synthesied
  misc_feature (1)..(10): P7-index
attcgccaac

SEQ ID NO: 815 - DNA, 10 bp, Artificial Sequence
  Synthesied
  misc_feature (1)..(10): P7-index
tgagagtctt

SEQ ID NO: 816 - DNA, 10 bp, Artificial Sequence
  Synthesied
  misc_feature (1)..(10): P7-index
gccatagtcg

SEQ ID NO: 817 - DNA, 10 bp, Artificial Sequence
  Synthesied
  misc_feature (1)..(10): P7-index
accagtgcaa

SEQ ID NO: 818 - DNA, 10 bp, Artificial Sequence
  Synthesied
  misc_feature (1)..(10): P7-index
tgagaccatt

SEQ ID NO: 819 - DNA, 10 bp, Artificial Sequence
  Synthesied
  misc_feature (1)..(10): P7-index
gatctatgcc

SEQ ID NO: 820 - DNA, 10 bp, Artificial Sequence
  Synthesied
  misc_feature (1)..(10): P7-index
ctgtcgatgg

SEQ ID NO: 821 - DNA, 10 bp, Artificial Sequence
  Synthesied
  misc_feature (1)..(10): P7-index
tatcgccgaa

SEQ ID NO: 822 - DNA, 10 bp, Artificial Sequence
  Synthesied
  misc_feature (1)..(10): P7-index
gtaattgctc

SEQ ID NO: 823 - DNA, 10 bp, Artificial Sequence
  Synthesied
  misc_feature (1)..(10): P7-index
acgtcgaagt

SEQ ID NO: 824 - DNA, 10 bp, Artificial Sequence
  Synthesied
  misc_feature (1)..(10): P7-index
cgcgaattcg

SEQ ID NO: 825 - DNA, 10 bp, Artificial Sequence
  Synthesied
  misc_feature (1)..(10): P7-index
ctgcttgtcc

SEQ ID NO: 826 - DNA, 10 bp, Artificial Sequence
  Synthesied
  misc_feature (1)..(10): P7-index
aataggcgtg

SEQ ID NO: 827 - DNA, 10 bp, Artificial Sequence
  Synthesied
  misc_feature (1)..(10): P7-index
tgatacacga

SEQ ID NO: 828 - DNA, 10 bp, Artificial Sequence
  Synthesied
  misc_feature (1)..(10): P7-index
gccgcataat

SEQ ID NO: 829 - DNA, 10 bp, Artificial Sequence
  Synthesied
  misc_feature (1)..(10): P7-index
ttcagtgcgg

SEQ ID NO: 830 - DNA, 10 bp, Artificial Sequence
  Synthesied
  misc_feature (1)..(10): P7-index
agagcaattc

SEQ ID NO: 831 - DNA, 10 bp, Artificial Sequence
  Synthesied
  misc_feature (1)..(10): P7-index
ccttagtaca

SEQ ID NO: 832 - DNA, 10 bp, Artificial Sequence
  Synthesied
  misc_feature (1)..(10): P7-index
gagctccgat

SEQ ID NO: 833 - DNA, 10 bp, Artificial Sequence
  Synthesied
  misc_feature (1)..(10): P7-index
catagcgagg

SEQ ID NO: 834 - DNA, 10 bp, Artificial Sequence
  Synthesied
  misc_feature (1)..(10): P7-index
atatcgtgct

SEQ ID NO: 835 - DNA, 10 bp, Artificial Sequence
  Synthesied
  misc_feature (1)..(10): P7-index
tggcaactta

SEQ ID NO: 836 - DNA, 10 bp, Artificial Sequence
  Synthesied
  misc_feature (1)..(10): P7-index
gccgttacac

SEQ ID NO: 837 - DNA, 10 bp, Artificial Sequence
  Synthesied
  misc_feature (1)..(10): P7-index
agtcctgcaa

SEQ ID NO: 838 - DNA, 10 bp, Artificial Sequence
  Synthesied
  misc_feature (1)..(10): P7-index
tcaagacggc

SEQ ID NO: 839 - DNA, 10 bp, Artificial Sequence
  Synthesied
  misc_feature (1)..(10): P7-index
gagtagattg

SEQ ID NO: 840 - DNA, 10 bp, Artificial Sequence
  Synthesied
  misc_feature (1)..(10): P7-index
ctcgtctact

SEQ ID NO: 841 - DNA, 10 bp, Artificial Sequence
  Synthesied
  misc_feature (1)..(10): P7-index
accacagcgt

SEQ ID NO: 842 - DNA, 10 bp, Artificial Sequence
  Synthesied
  misc_feature (1)..(10): P7-index
caactcctac

SEQ ID NO: 843 - DNA, 10 bp, Artificial Sequence
  Synthesied
  misc_feature (1)..(10): P7-index
ttgtgtaacg

SEQ ID NO: 844 - DNA, 10 bp, Artificial Sequence
  Synthesied
  misc_feature (1)..(10): P7-index
ggtgagtgta

SEQ ID NO: 845 - DNA, 10 bp, Artificial Sequence
  Synthesied
  misc_feature (1)..(10): P7-index
tggttgcgca

SEQ ID NO: 846 - DNA, 10 bp, Artificial Sequence
  Synthesied
  misc_feature (1)..(10): P7-index
aacggtattg

SEQ ID NO: 847 - DNA, 10 bp, Artificial Sequence
  Synthesied
  misc_feature (1)..(10): P7-index
gtacaagcac

SEQ ID NO: 848 - DNA, 10 bp, Artificial Sequence
  Synthesied
  misc_feature (1)..(10): P7-index
cctacctagt

SEQ ID NO: 849 - DNA, 10 bp, Artificial Sequence
  Synthesied
  misc_feature (1)..(10): P7-index
agatcgctgg

SEQ ID NO: 850 - DNA, 10 bp, Artificial Sequence
  Synthesied
  misc_feature (1)..(10): P7-index
cctcacaaca

SEQ ID NO: 851 - DNA, 10 bp, Artificial Sequence
  Synthesied
  misc_feature (1)..(10): P7-index
taggtatcac

SEQ ID NO: 852 - DNA, 10 bp, Artificial Sequence
  Synthesied
  misc_feature (1)..(10): P7-index
gtcagtggtt